European Patent Specification EP 3 456 826 B1, published June 28, 2023. Title: TAL EFFECTOR-MEDIATED DNA MODIFICATION. Applicant: Regents of the University of Minnesota Iowa State University Research Foundation, Inc. Application PCT/US2010/059932. The sequence listing filed with the application follows.

SEQUENCE LISTING (93 sequences)

SEQ ID NO: 1 - protein, 34 aa, Artificial Sequence
  generic sequence
LTPDQVVAIASHDGGKQALETVQRLLPVLCQAHG

SEQ ID NO: 2 - DNA, 17 bp, Artificial Sequence
  target sequence
agaagaagagacccata

SEQ ID NO: 3 - DNA, 18 bp, Artificial Sequence
  target sequence
atataaacctaaccatcc

SEQ ID NO: 4 - DNA, 18 bp, Artificial Sequence
  target sequence
atataaacctgacccttt

SEQ ID NO: 5 - DNA, 14 bp, Artificial Sequence
  target sequence
atataaacctctct

SEQ ID NO: 6 - DNA, 15 bp, Artificial Sequence
  target sequence
atataaacctaacca

SEQ ID NO: 7 - DNA, 14 bp, Artificial Sequence
  target sequence
ataaacctaaccat

SEQ ID NO: 8 - DNA, 24 bp, Artificial Sequence
  target sequence
gcatctccccctactgtacaccac

SEQ ID NO: 9 - DNA, 23 bp, Artificial Sequence
  target sequence
ataaaaggccctcaccaacccat

SEQ ID NO: 10 - DNA, 22 bp, Artificial Sequence
  target sequence
ataatccccaaatcccctcctc

SEQ ID NO: 11 - DNA, 16 bp, Artificial Sequence
  target sequence
ccccctcgcttccctt

SEQ ID NO: 12 - protein, 1164 aa, Xanthomonas euvesicatoria
MDPIRSRTPSPARELLPGPQPDGVQPTADRGVSPPAGGPLDGLPARRTMSRTRLPSPPAPSPAFSAGSFSDLLRQFDPSLFNTSLFDSLPPFGAHHTEAATGEWDEVQSGLRAADAPPPTMRVAVTAARPPRAKPAPRRRAAQPSDASPAAQVDLRTLGYSQQQQEKIKPKVRSTVAQHHEALVGHGFTHAHIVALSQHPAALGTVAVKYQDMIAALPEATHEAIVGVGKQWSGARALEALLTVAGELRGPPLQLDTGQLLKIAKRGGVTAVEAVHAWRNALTGAPLNLTPEQVVAIASHDGGKQALETVQRLLPVLCQAHGLTPQQVVAIASNGGGKQALETVQRLLPVLCQAHGLTPQQVVAIASNSGGKQALETVQRLLPVLCQAHGLTPEQVVAIASNGGGKQALETVQRLLPVLCQAHGLTPEQVVAIASNIGGKQALETVQALLPVLCQAHGLTPEQVVAIASNIGGKQALETVQALLPVLCQAHGLTPEQVVAIASNIGGKQALETVQALLPVLCQAHGLTPEQVVAIASHDGGKQALETVQRLLPVLCQAHGLTPEQVVAIASHDGGKQALETVQRLLPVLCQAHGLTPQQVVAIASNGGGKQALETVQRLLPVLCQAHGLTPEQVVAIASNSGGKQALETVQALLPVLCQAHGLTPEQVVAIASNSGGKQALETVQRLLPVLCQAHGLTPEQVVAIASHDGGKQALETVQRLLPVLCQAHGLTPEQVVAIASHDGGKQALETVQRLLPVLCQAHGLTPEQVVAIASHDGGKQALETVQRLLPVLCQAHGLTPQQVVAIASNGGGRPALETVQRLLPVLCQAHGLTPEQVVAIASHDGGKQALETVQRLLPVLCQAHGLTPQQVVAIASNGGGRPALESIVAQLSRPDPALAALTNDHLVALACLGGRPALDAVKKGLPHAPALIKRTNRRIPERTSHRVADHAQVVRVLGFFQCHSHPAQAFDDAMTQFGMSRHGLLQLFRRVGVTELEARSGTLPPASQRWDRILQASGMKRAKPSPTSTQTPDQASLHAFADSLERDLDAPSPMHEGDQTRASSRKRSRSDRAVTGPSAQQSFEVRVPEQRDALHLPLSWRVKRPRTSIGGGLPDPGTPTAADLAASSTVMREQDEDPFAGAADDFPAFNEEELAWLMELLPQ

SEQ ID NO: 13 - DNA, 4366 bp, Xanthomonas euvesicatoria
gaattcaaggtgtcaaaaagcgataggcggaattatagatgtacttgtatgaacttatcaacgccagtttagtgaacgggttcgacaaagcgaaaccaacacccaggcgcgaaagccttgcgccgcaatgctttccggcaatgtgacccagggcattgaccgaaacggcgtaggaatttcggaacacgacggtaggggaatgctctaccgcccggctacgcaaaagcactctcgcctgccagacgcgccactgcgtggaattggccgttatgtccgctggcggcctcgccgccgtagtgcttgcagcgcagccttgaatgatcgaacatcaaacatcactgtttgataggtcgatcatgacatcgcccatttcgagggtcggcagggattcgtgtaaaaaacagccaaaagtgagctaactcgctgtcagcacagaaatttttcacaaccttctgccgatcctccatgcgggtccgtgatcgccttcatgtctgcgcctcaccctggtcgtcgagggttgccaggatcacccgaagttgtgtactgccatgcggcctcggaagctatgtaggaaccacagaccgctagtctggaggcgaccatgtaaagaggtatgcctgatggatcccattcgttcgcgcacaccaagtcctgcccgcgagcttctgcccggaccccaacccgatggggttcagccgactgcagatcgtggggtgtctccgcctgccggcggccccctggatggcttgcccgctcggcggacgatgtcccggacccggctgccatctccccctgccccctcacctgcgttctcggcgggcagcttcagtgacctgttacgtcagttcgatccgtcactttttaatacatcgctttttgattcattgcctcccttcggcgctcaccatacagaggctgccacaggcgagtgggatgaggtgcaatcgggtctgcgggcagccgacgcccccccacccaccatgcgcgtggctgtcactgccgcgcggccgccgcgcgccaagccggcgccgcgacgacgtgctgcgcaaccctccgacgcttcgccggccgcgcaggtggatctacgcacgctcggctacagccagcagcaacaggagaagatcaaaccgaaggttcgttcgacagtggcgcagcaccacgaggcactggtcggccatgggtttacacacgcgcacatcgttgcgctcagccaacacccggcagcgttagggaccgtcgctgtcaagtatcaggacatgatcgcagcgttgccagaggcgacacacgaagcgatcgttggcgtcggcaaacagtggtccggcgcacgcgctctggaggccttgctcacggtggcgggagagttgagaggtccaccgttacagttggacacaggccaacttctcaagattgcaaaacgtggcggcgtgaccgcagtggaggcagtgcatgcatggcgcaatgcactgacgggtgcccccctgaacctgaccccggagcaggtggtggccatcgccagccacgatggcggcaagcaggcgctggagacggtgcagcggctgttgccggtgctgtgccaggcccatggcctgaccccgcagcaggtggtggccatcgccagcaatggcggtggcaagcaggcgctggagacggtgcagcggctgttgccggtgctgtgccaggcccatggcctgaccccgcagcaggtggtggccatcgccagcaatagcggtggcaagcaggcgctggagacggtgcagcggctgttgccggtgctgtgccaggcccatggcctgaccccggagcaggtggtggccatcgccagcaatggcggtggcaagcaggcgctggagacggtgcagcggctgttgccggtgctgtgccaggcccatggcctgaccccggagcaggtggtggccatcgccagcaatattggtggcaagcaggcgctggagacggtgcaggcgctgttgccggtgctgtgccaggcccatggcctgaccccggagcaggtggtggccatcgccagcaatattggtggcaagcaggcgctggagacggtgcaggcgctgttgccggtgctgtgccaggcccatggcctgaccccggagcaggtggtggccatcgccagcaatattggtggcaagcaggcgctggagacggtgcaggcgctgttgccggtgctgtgccaggcccatggcctgaccccggagcaggtggtggccatcgccagccacgatggcggcaagcaggcgctggagacggtgcagcggctgttgccggtgctgtgccaggcccatggcctgaccccggagcaggtggtggccatcgccagccacgatggcggcaagcaggcgctggagacggtgcagcggctgttgccggtgctgtgccaggcccatggcctgaccccgcagcaggtggtggccatcgccagcaatggcggtggcaagcaggcgctggagacggtgcagcggctgttgccggtgctgtgccaggcccatggcctgaccccggagcaggtggtggccatcgccagcaatagcggtggcaagcaggcgctggagacggtgcaggcgctgttgccggtgctgtgccaggcccatggcctgaccccggagcaggtggtggccatcgccagcaatagcggtggcaagcaggcgctggagacggtgcagcggctgttgccggtgctgtgccaggcccatggcctgaccccggagcaggtggtggccatcgccagccacgatggcggcaagcaggcgctggagacggtgcagcggctgttgccggtgctgtgccaggcccatggcctgaccccggagcaggtggtggccatcgccagccacgatggcggcaagcaggcgctggagacggtgcagcggctgttgccggtgctgtgccaggcccatggcctgaccccggagcaggtggtggccatcgccagccacgatggcggcaagcaggcgctggagacggtgcagcggctgttgccggtgctgtgccaggcccatggcctgaccccgcagcaggtggtggccatcgccagcaatggcggcggcaggccggcgctggagacggtgcagcggctgttgccggtgctgtgccaggcccatggcctgaccccggagcaggtggtggccatcgccagccacgatggcggcaagcaggcgctggagacggtgcagcggctgttgccggtgctgtgccaggcccatggcctgaccccgcagcaggtggtggccatcgccagcaatggcggcggcaggccggcgctggagagcattgttgcccagttatctcgccctgatccggcgttggccgcgttgaccaacgaccacctcgtcgccttggcctgcctcggcggacgtcctgcgctggatgcagtgaaaaagggattgccgcacgcgccggccttgatcaaaagaaccaatcgccgtattcccgaacgcacatcccatcgcgttgccgaccacgcgcaagtggttcgcgtgctgggttttttccagtgccactcccacccagcgcaagcatttgatgacgccatgacgcagttcgggatgagcaggcacgggttgttacagctctttcgcagagtgggcgtcaccgaactcgaagcccgcagtggaacgctccccccagcctcgcagcgttgggaccgtatcctccaggcatcagggatgaaaagggccaaaccgtcccctacttcaactcaaacgccggatcaggcgtctttgcatgcattcgccgattcgctggagcgtgaccttgatgcgcctagcccaatgcacgagggagatcagacgcgggcaagcagccgtaaacggtcccgatcggatcgtgctgtcaccggtccctccgcacagcaatcgttcgaggtgcgcgttcccgaacagcgcgatgcgctgcatttgcccctcagttggagggtaaaacgcccgcgtaccagtatcgggggcggcctcccggatcctggtacgcccacggctgccgacctggcagcgtccagcaccgtgatgcgggaacaagatgaggaccccttcgcaggggcagcggatgatttcccggcattcaacgaagaggagctcgcatggttgatggagctattgcctcagtgaggctcagtcggtgactacctgagcgtcggcagggattggtgtaagtaacctttactgacagcgagttagcccacttttggctgttttttacacaaatccctgcctcccctctggttgcaccacacccgtacaccaagcgcggcggcgaagcaggcaccgagtggttccgctgcggtgttgcgttccctaaccagggcggtggctatacgctcaagctgcgcaccgtcccggtggcgatcgacgacgaaatg

SEQ ID NO: 14 - DNA, 56 bp, Artificial Sequence
  target sequence
tatataaacctaaccatcctcacaacttcaagttatcggatggttaggtttatata

SEQ ID NO: 15 - DNA, 56 bp, Artificial Sequence
  target sequence
tatataaacctaaccatccgataacttgaagttgtgaggatggttaggtttatata

SEQ ID NO: 16 - protein, 1373 aa, Xanthomonas euvesicatoria
MDPIRSRTPSPARELLPGPQPDRVQPTADRGGAPPAGGPLDGLPARRTMSRTRLPSPPAPSPAFSAGSFSDLLRQFDPSLLDTSLLDSMPAVGTPHTAAAPAECDEVQSGLRAADDPPPTVRVAVTAARPPRAKPAPRRRAAQPSDASPAAQVDLRTLGYSQQQQEKIKPKVGSTVAQHHEALVGHGFTHAHIVALSRHPAALGTVAVKYQDMIAALPEATHEDIVGVGKQWSGARALEALLTVAGELRGPPLQLDTGQLVKIAKRGGVTAVEAVHASRNALTGAPLNLTPAQVVAIASNNGGKQALETVQRLLPVLCQAHGLTPAQVVAIASHDGGKQALETMQRLLPVLCQAHGLPPDQVVAIASNIGGKQALETVQRLLPVLCQAHGLTPDQVVAIASHGGGKQALETVQRLLPVLCQAHGLTPDQVVAIASHDGGKQALETVQRLLPVLCQAHGLTPDQVVAIASNGGGKQALETVQRLLPVLCQAHGLTPDQVVAIASNGGKQALETVQRLLPVLCQAHGLTPDQVVAIASHDGGKQALETVQRLLPVLCQTHGLTPAQVVAIASHDGGKQALETVQQLLPVLCQAHGLTPDQVVAIASNIGGKQALATVQRLLPVLCQAHGLTPDQVVAIASNGGGKQALETVQRLLPVLCQAHGLTPDQVVAIASNGGGKQALETVQRLLPVLCQAHGLTQVQVVAIASNIGGKQALETVQRLLPVLCQAHGLTPAQVVAIASHDGGKQALETVQRLLPVLCQAHGLTPDQVVAIASNGGGKQALETVQRLLPVLCQAHGLTQEQVVAIASNNGGKQALETVQRLLPVLCQAHGLTPDQVVAIASNGGGKQALETVQRLLPVLCQAHGLTPAQVVAIASNIGGKQALETVQRLLPVLCQDHGLTLAQVVAIASNIGGKQALETVQRLLPVLCQAHGLTQDQVVAIASNIGGKQALETVQRLLPVLCQDHGLTPDQVVAIASNIGGKQALETVQRLLPVLCQDHGLTLDQVVAIASNGGKQALETVQRLLPVLCQDHGLTPDQVVAIASNSGGKQALETVQRLLPVLCQDHGLTPNQVVAIASNGGKQALESIVAQLSRPDPALAALTNDHLVALACLGGRPAMDAVKKGLPHAPELIRRVNRRIGERTSHRVADYAQVVRVLEFFQCHSHPAYAFDEAMTQFGMSRNGLVQLFRRVGVTELEARGGTLPPASQRWDRILQASGMKRAKPSPTSAQTPDQASLHAFADSLERDLDAPSPMHEGDQTGASSRKRSRSDRAVTGPSAQHSFEVRVPEQRDALHLPLSWRVKRPRTRIGGGLPDPGTPIAADLAASSTVMWEQDAAPFAGAADDFPAFNEEELAWLMELLPQSGSVGGTI

SEQ ID NO: 17 - DNA, 102 bp, Artificial Sequence
  synthetic
  misc_feature 34, 35, 36: n = CAT or CAC or AAC or AAT
  misc_feature 37, 38, 39: n = GAC or GAT or GGA or GGC or GGG or GGT or TCA or TCC or TCG or TCT or AGC or AGT or ATA or ATC or ATT
ctgaccccggcacaggtggtggccatcgccagcnnnnnnggcggcaagcaggcgctggagacggtgcagcggctgttgccggtgctgtgccaggaccatggc

SEQ ID NO: 18 - protein, 34 aa, Artificial Sequence
  synthetic
  VARIANT 12, 13: Xaa = His Asp or Asn Gly or Asn Ser or Asn Ile
LTPAQVVAIASXXGGKQALETVQRLLPVLCQDHG

SEQ ID NO: 19 - DNA, 63 bp, Artificial Sequence
  synthetic
  misc_feature 34, 35, 36: n = CAT or CAC or AAC or AAT
  misc_feature 37, 38, 39: n = GAC or GAT or GGA or GGC or GGG or GGT or TCA or TCC or TCG or TCT or AGC or AGT or ATA or ATC or ATT
ctgaccccggcacaggtggtggccatcgccagcnnnnnnggcggcaagcaggcgctcgagagc

SEQ ID NO: 20 - protein, 21 aa, Artificial Sequence
  synthetic
  VARIANT 12, 13: Xaa = His Asp or Asn Gly or Asn Ser or Asn Ile
LTPAQVVAIASXXGGKQALES

SEQ ID NO: 21 - DNA, 12 bp, Xanthomonas oryzae
gcgctggagagc

SEQ ID NO: 22 - protein, 4 aa, Xanthomonas oryzae
ALES

SEQ ID NO: 23 - DNA, 12 bp, Artificial Sequence
  synthetic
gcgctcgagtcc

SEQ ID NO: 24 - DNA, 102 bp, Artificial Sequence
  synthetic
tcgagacggtgcagcggctgttgccggtgctgtgccaggaccatggcctgaccccggaccaagtggtggccatcgccagcaacattggcggcaagcaagcgc

SEQ ID NO: 25 - DNA, 102 bp, Artificial Sequence
  synthetic
tcgagcgcttgcttgccgccaatgttgctggcgatggccaccacttggtccggggtcaggccatggtcctggcacagcaccggcaacagccgctgcaccgtc

SEQ ID NO: 26 - protein, 35 aa, Artificial Sequence
  synthetic
ETVQRLLPVLCQDHGLTPDQVVAIASNIGGKQALE

SEQ ID NO: 27 - DNA, 102 bp, Artificial Sequence
  synthetic
tcgaaacggtgcagcggctgttgccggtgctgtgccaggaccatggcctgaccccggaccaagtggtggctatcgccagcaacattggcggcaagcaagcgc

SEQ ID NO: 28 - DNA, 102 bp, Artificial Sequence
  synthetic
tcgagcgcttgcttgccgccaatgttgctggcgatagccaccacttggtccggggtcaggccatggtcctggcacagcaccggcaacagccgctgcaccgtt

SEQ ID NO: 29 - DNA, 18 bp, Artificial Sequence
  target sequence
atcaagattctcttcact

SEQ ID NO: 30 - DNA, 15 bp, Artificial Sequence
  target sequence
cccagaagtaaacat

SEQ ID NO: 31 - protein, 598 aa, Xanthomonas oryzae
LTPEQVVAIASHDGGKQALETVQRLLPVLCQAHGLTPQQVVAIASNGGGKQALETVQRLLPVLCQAHGLTPQQVVAIASNSGGKQALETVQRLLPVLCQAHGLTPEQVVAIASNGGGKQALETVQRLLPVLCQAHGLTPEQVVAIASNIGGKQALETVQALLPVLCQAHGLTPEQVVAIASNIGGKQALETVQALLPVLCQAHGLTPEQVVAIASNIGGKQALETVQALLPVLCQAHGLTPEQVVAIASHDGGKQALETVQRLLPVLCQAHGLTPEQVVAIASHDGGKQALETVQRLLPVLCQAHGLTPQQVVAIASNGGGKQALETVQRLLPVLCQAHGLTPEQVVAIASNSGGKQALETVQALLPVLCQAHGLTPEQVVAIASNSGGKQALETVQRLLPVLCQAHGLTPEQVVAIASHDGGKQALETVQRLLPVLCQAHGLTPEQVVAIASHDGGKQALETVQRLLPVLCQAHGLTPEQVVAIASHDGGKQALETVQRLLPVLCQAHGLTPQQVVAIASNGGGRPALETVQRLLPVLCQAHGLTPEQVVAIASHDGGKQALETVQRLLPVLCQAHGLTPQQVVAIASNGGGRPALE

SEQ ID NO: 32 - DNA, 4122 bp, Xanthomonas oryzae
atggatcccattcgttcgcgcacgccaagtcctgcccgcgagcttctgcccggaccccaaccggatagggttcagccgactgcagatcgggggggggctccgcctgctggcggccccctggatggcttgcccgctcggcggacgatgtcccggacccggctgccatctccccctgcgccctcgcctgcgttctcggcgggcagcttcagcgatctgctccgtcagttcgatccgtcgcttcttgatacatcgcttcttgattcgatgcctgccgtcggcacgccgcatacagcggctgccccagcagagtgcgatgaggtgcaatcgggtctgcgtgcagccgatgacccgccacccaccgtgcgtgtcgctgtcactgccgcgcggccgccgcgcgccaagccggccccgcgacggcgtgcggcgcaaccctccgacgcttcgccggccgcgcaggtggatctacgcacgctcggctacagtcagcagcagcaagagaagatcaaaccgaaggtgggttcgacagtggcgcagcaccacgaggcactggtgggccatgggtttacacacgcgcacatcgttgcgctcagccgacacccggcagcgttagggaccgtcgctgtcaagtatcaggacatgatcgcggcgttaccagaggcgacacacgaagacatcgttggtgtcggcaaacagtggtccggcgcacgcgccctggaggccttgctcacggtggcgggagagttgagaggtccaccgttacagttggacacaggccaacttgtcaagattgcaaaacgtggcggcgtgaccgcagtggaggcagtgcatgcatcgcgcaatgcactgacgggtgcccccctgaacctgaccccggcacaggtggtggccatcgccagcaataacggtggcaagcaggcgctggagacggtgcagcggctgttgccggtgctgtgccaggcccatggcctgaccccggcgcaggtggtggccatcgccagccacgatggcggcaagcaggcactggagacgatgcagcggctgttgccggtgctgtgccaggcccatggcctgcccccggaccaggtggtggccatcgccagcaatattggcggcaagcaggcgctggagacggtgcagcggctgttgccggtgctctgccaggcccatggcctgaccccggaccaggtggtggccatcgccagccatggcggcggcaagcaggcgctggagacggtgcagcggctgttgccggtgctctgccaggcccatggcctgaccccggaccaggtggtggccatcgccagccacgatggcggcaagcaggcgctggagacggtgcagcggctgttgccggtgctgtgccaggcccatggcctgaccccggaccaggtggtggccatcgccagcaatggcggcggcaagcaggcgctggagacggtgcagcggctgttgccggtgctgtgccaggcccatggtctgaccccggaccaggtggtggccatcgccagcaatggcggcaagcaggcgctggagacggtgcagcggctgttgccggtgctgtgccaggcccatggcctgaccccggaccaggtggtggccatcgccagccacgatggcggcaagcaggcgctggagacggtgcagcggctgttgccggtgctgtgccagacccatggtctgaccccggcgcaggtggtggccatcgccagccacgatggcggcaagcaggcgctggagacggtgcagcagctgttgccggtgctgtgccaggcccatggcctgaccccggaccaggtggtggccatcgccagcaatattggcggcaagcaggcgctagcgacggtgcagcggctgttgccggtgctgtgccaagcccatggcctgaccccggaccaggtggtggccatcgccagcaatggcggcggcaagcaggcgctggagacggtgcagcggctgttgccggtgctgtgccaggcccatggcctgaccccggaccaggtggtggccatcgccagcaatggcggcggcaagcaggcgctggagacggtgcagcggctgttgccggtgctgtgccaggcccatggtctgacccaggtgcaggtggtggccatcgccagcaatattggcggcaagcaggcgctggagacggtgcagcggctgttgccggtgctgtgccaggcccatggcctgaccccggcgcaggtggtggccatcgccagccacgatggcggcaagcaggcgctggagacggtgcagcggctgttgccggtgctgtgccaggcccatggcctgaccccggaccaagtggtggccatcgccagcaatggcggcggcaagcaggcgctggagacggtgcagcggctgttgccggtgctgtgccaggcccatggcctgacccaggagcaggtggtggccatcgccagcaataacggcggcaagcaggcgctggagacggtgcagcggctgttgccggtgctgtgccaggcccatggcctgaccccggaccaggtggtggccatcgccagcaatggcggcggcaagcaggcgctggagacggtgcagcggctgttgccggtgctgtgccaggcccatggtctgaccccggcgcaggtggtggccatcgccagcaatattggcggcaagcaggcgctggagacggtgcagcggctgttgccggtgctgtgccaggaccatggcctgaccctggcgcaggtggtggccatcgccagcaatattggcggcaagcaggcgctggagacggtgcagcggctgttgccggtgctgtgccaggcacatggcctgacccaggaccaggtggtggccatcgccagcaatattggcggcaagcaggcgctggagacggtgcagcggctgttgccggtgctgtgccaggaccatggcctgaccccggaccaggtcgtggccatcgccagcaatattggcggcaagcaggcgctggagacggtgcagcggctgttgccggtgctgtgccaggaccatggcctgaccctggaccaggtggtggccatcgccagcaatggcggcaagcaggcgctggagacggtgcagcggctgttgccggtgctgtgccaggaccatggactgaccccggaccaggtcgtggccatcgccagcaatagtggcggcaagcaggcgctggagacggtgcagcggctgttgccggtgctgtgccaggaccatggcctgaccccgaaccaggtggtggccatcgccagcaatggcggcaagcaggcgctggagagcattgttgcccagttatctcgccctgatccggcgttggccgcgttgaccaacgaccacctcgtcgccttggcctgcctcggcggacgtcctgccatggatgcagtgaaaaagggattgccgcacgcgccggaattgatcagaagagtcaatcgccgtattggcgaacgcacgtcccatcgcgttgccgactacgcgcaagtggttcgcgtgctggagtttttccagtgccactcccacccagcgtacgcatttgatgaggccatgacgcagttcgggatgagcaggaacgggttggtacagctctttcgcagagtgggcgtcaccgaactcgaagcccgcggtggaacgctccccccagcctcgcagcgttgggaccgtatcctccaggcatcagggatgaaaagggccaaaccgtcccctacttcagctcaaacaccggatcaggcgtctttgcatgcattcgccgattcgctggagcgtgaccttgatgcgcctagcccaatgcacgagggagatcagacaggggcaagcagccgtaaacggtcccgatcggatcgtgctgtcaccggcccctccgcacagcactctttcgaggtgcgcgttcccgaacagcgcgatgcgctgcatttgcccctcagctggagggtaaaacgcccgcgtaccaggatcgggggcggcctcccggatcctggtacgcccatcgctgccgacctggcagcgtccagcaccgtgatgtgggaacaagatgcggcccccttcgcaggggcagcggatgatttcccggcattcaacgaagaggagctcgcatggttgatggagctattgcctcagtcaggctcagtcggagggacgatctga

SEQ ID NO: 33 - protein, 1341 aa, Artificial Sequence
  synthetic
MASSPPKKKRKVSWKDASGWSRMHADPIRSRTPSPARELLPGPQPDGVQPTADRGVSPPAGGPLDGLPARRTMSRTRLPSPPAPSPAFSAGSFSDLLRQFDPSLFNTSLFDSLPPFGAHHTEAATGEWDEVQSGLRAADAPPPTMRVAVTAARPPRAKPAPRRRAAQPSDASPAAQVDLRTLGYSQQQQEKIKPKVRSTVAQHHEALVGHGFTHAHIVALSQHPAALGTVAVKYQDMIAALPEATHEAIVGVGKQWSGARALEALLTVAGELRGPPLQLDTGQLLKIAKRGGVTAVEAVHAWRNALTGAPLNLTPEQVVAIASHDGGKQALETVQRLLPVLCQAHGLTPQQVVAIASNGGGKQALETVQRLLPVLCQAHGLTPQQVVAIASNSGGKQALETVQRLLPVLCQAHGLTPEQVVAIASNGGGKQALETVQRLLPVLCQAHGLTPEQVVAIASNIGGKQALETVQALLPVLCQAHGLTPEQVVAIASNIGGKQALETVQALLPVLCQAHGLTPEQVVAIASNIGGKQALETVQALLPVLCQAHGLTPEQVVAIASHDGGKQALETVQRLLPVLCQAHGLTPEQVVAIASHDGGKQALETVQRLLPVLCQAHGLTPQQVVAIASNGGGKQALETVQRLLPVLCQAHGLTPEQVVAIASNSGGKQALETVQALLPVLCQAHGLTPEQVVAIASNSGGKQALETVQRLLPVLCQAHGLTPEQVVAIASHDGGKQALETVQRLLPVLCQAHGLTPEQVVAIASHDGGKQALETVQRLLPVLCQAHGLTPEQVVAIASHDGGKQALETVQRLLPVLCQAHGLTPQQVVAIASNGGGRPALETVQRLLPVLCQAHGLTPEQVVAIASHDGGKQALETVQRLLPVLCQAHGLTPQQVVAIASNGGGRPALESIVAQLSRPDPALAALTNDHLVALACLGGRPALDAVKKGLPHAPALIKRTNRRIPERTSHRVADHAQVVRVLGFFQCHSHPAQAFDDAMTQFGMSRHGLLQLFRRVGVTELEARSGTLPPASQRWDRILQASGMKRAKPSPTSTQTPDQASLHAFADSLERDLDAPSPMHEGDQTRASSRKRSRSDRAVTGPSAQQSFEVRVPEQRDALHLPLSWRVKRPRTSIGGGLPDPISRSQLVKSELEEKKSELRHKLKYVPHEYIELIEIARNSTQDRILEMKVMEFFMKVYGYRGKHLGGSRKPDGAIYTVGSPIDYGVIVDTKAYSGGYNLPIGQADEMQRYVEENQTRNKHINPNEWWKVYPSSVTEFKFLFVSGHFKGNYKAQLTRLNHITNCNGAVLSVEELLIGGEMIKAGTLTLEEVRRKFNNGEINF

SEQ ID NO: 34 - protein, 1542 aa, Artificial Sequence
  synthetic
MASSPPKKKRKVSWKDASGWSRMHADPIRPRRPSPARELLPGPQPDRVQPTADRGVSAPAGSPLDGLPARRTVSRTRLPSPPAPSPAFSAGSFSDLLRPFDPSLLDTSLLDSMPAVGTPHTAAAPAEWDEAQSALRAADDPPPTVRVAVTAARPPRAKPAPRRRAAQPSDASPAAQVDLRTLGYSQQQQEKIKPKVRSTVAQHHEALVGHGFTHAHIVALSQHPAALGTVAVTYQHIITALPEATHEDIVGVGKQWSGARALEALLTDAGELRGPPLQLDTGQLVKIAKRGGVTAMEAVHASRNALTGAPLNLTPAQVVAIASNNGGKQALETVQRLLPVLCQAHGLTPAQVVAIASHDGGKQALETMQRLLPVLCQAHGLPPDQVVAIASNIGGKQALETVQRLLPVLCQAHGLTPDQVVAIASHGGGKQALETVQRLLPVLCQAHGLTPDQVVAIASHDGGKQALETVQRLLPVLCQAHGLTPDQVVAIASNGGGKQALETVQRLLPVLCQAHGLTPDQVVAIASNGGKQALETVQRLLPVLCQAHGLTPDQVVAIASHDGGKQALETVQRLLPVLCQTHGLTPAQVVAIASHDGGKQALETVQQLLPVLCQAHGLTPDQVVAIASNIGGKQALATVQRLLPVLCQAHGLTPDQVVAIASNGGGKQALETVQRLLPVLCQAHGLTPDQVVAIASNGGGKQALETVQRLLPVLCQAHGLTQVQVVAIASNIGGKQALETVQRLLPVLCQAHGLTPAQVVAIASHDGGKQALETVQRLLPVLCQAHGLTPDQVVAIASNGGGKQALETVQRLLPVLCQAHGLTQEQVVAIASNNGGKQALETVQRLLPVLCQAHGLTPDQVVAIASNGGGKQALETVQRLLPVLCQAHGLTPAQVVAIASNIGGKQALETVQRLLPVLCQDHGLTLAQVVAIASNIGGKQALETVQRLLPVLCQAHGLTQDQVVAIASNIGGKQALETVQRLLPVLCQDHGLTPDQVVAIASNIGGKQALETVQRLLPVLCQDHGLTLDQVVAIASNGGKQALETVQRLLPVLCQDHGLTPDQVVAIASNSGGKQALETVQRLLPVLCQDHGLTPNQVVAIASNGGKQALESIVAQLSRPDPALAALTNDHLVALACLGGRPAMDAVKKGLPHAPELIRRVNRRIGERTSHRVADYAQVVRVLEFFQCHSHPAYAFDEAMTQFGMSRNGLVQLFRRVGVTELEARGGTLPPASQRWDRILQASGMKRAKPSPTSAQTPDQASLHAFADSLERDLDAPSPMHEGDQTRASSRKRSRSDRAVTGPSAQQAVEVRVPEQRDALHLPLSWRVKRPRTRIWGGLPDPISRSQLVKSELEEKKSELRHKLKYVPHEYIELIEIARNSTQDRILEMKVMEFFMKVYGYRGKHLGGSRKPDGAIYTVGSPIDYGVIVDTKAYSGGYNLPIGQADEMQRYVEENQTRNKHINPNEWWKVYPSSVTEFKFLFVSGHFKGNYKAQLTRLNHITNCNGAVLSVEELLIGGEMIKAGTLTLEEVRRKFNNGEINF

SEQ ID NO: 35 - protein, 1035 aa, Artificial Sequence
  synthetic
MASSPPKKKRKVSWKDASGWSRMHADPIRPRRPSPARELLPGPQPDRVQPTADRGVSAPAGSPLDGLPARRTVSRTRLPSPPAPSPAFSAGSFSDLLRPFDPSLLDTSLLDSMPAVGTPHTAAAPAEWDEAQSALRAADDPPPTVRVAVTAARPPRAKPAPRRRAAQPSDASPAAQVDLRTLGYSQQQQEKIKPKVRSTVAQHHEALVGHGFTHAHIVALSQHPAALGTVAVTYQHIITALPEATHEDIVGVGKQWSGARALEALLTDAGELRGPPLQLDTGQLVKIAKRGGVTAMEAVHASRNALTGAPLNLTPAQVVAIASHDGGKQALETVQRLLPVLCQDHGLTPDQVVAIANNNGGKQALETVQRLLPVLCQDHGLTPDQVVAIANNNGGKQALETVQRLLPVLCQDHGLTPDQVVAIASNGGGKQALETVQRLLPVLCQDHGLTPDQVVAIASNGGGKQALETVQRLLPVLCQDHGLTPDQVVAIASNGGGKQALETVQRLLPVLCQDHGLTPDQVVAIANNNGGKQALETVQRLLPVLCQDHGLTPDQVVAIASHDGGKQALETVQRLLPVLCQDHGLTPDQVVAIASNGGGKQALESIVAQLSRRDPALAALTNDHLVALACLGGRPALDAVKKGLPHAPEFIRRVNRRIAERTSHRVADYAHVVRVLEFFQCHSHPAHAFDEAMTQFGMSRHGLVQLFRRVGVTEFEARYGTLPPASQRWDRILQASGMKRAKPSPTSAQTPDQTSLHAFADSLERDLDAPSPMHEGDQTRASSRKRSRSDRAVTGPSAQQAVEVRVPEQRDALHLPLSWRVKRPRTRIWGGLPDPISRSQLVKSELEEKKSELRHKLKYVPHEYIELIEIARNSTQDRILEMKVMEFFMKVYGYRGKHLGGSRKPDGAIYTVGSPIDYGVIVDTKAYSGGYNLPIGQADEMQRYVEENQTRNKHINPNEWWKVYPSSVTEFKFLFVSGHFKGNYKAQLTRLNHITNCNGAVLSVEELLIGGEMIKAGTLTLEEVRRKFNNGEINF

SEQ ID NO: 36 - protein, 1069 aa, Artificial Sequence
  synthetic
MASSPPKKKRKVSWKDASGWSRMHADPIRPRRPSPARELLPGPQPDRVQPTADRGVSAPAGSPLDGLPARRTVSRTRLPSPPAPSPAFSAGSFSDLLRPFDPSLLDTSLLDSMPAVGTPHTAAAPAEWDEAQSALRAADDPPPTVRVAVTAARPPRAKPAPRRRAAQPSDASPAAQVDLRTLGYSQQQQEKIKPKVRSTVAQHHEALVGHGFTHAHIVALSQHPAALGTVAVTYQHIITALPEATHEDIVGVGKQWSGARALEALLTDAGELRGPPLQLDTGQLVKIAKRGGVTAMEAVHASRNALTGAPLNLTPAQVVAIASNIGGKQALETVQRLLPVLCQDHGLTPDQVVAIASHDGGKQALETVQRLLPVLCQDHGLTPDQVVAIASHDGGKQALETVQRLLPVLCQDHGLTPDQVVAIASHDGGKQALETVQRLLPVLCQDHGLTPDQVVAIASHDGGKQALETVQRLLPVLCQDHGLTPDQVVAIASNGGGKQALETVQRLLPVLCQDHGLTPDQVVAIASHDGGKQALETVQRLLPVLCQDHGLTPDQVVAIASNGGGKQALETVQRLLPVLCQDHGLTPDQVVAIASHDGGKQALETVQRLLPVLCQDHGLTPDQVVAIASHDGGKQALESIVAQLSRRDPALAALTNDHLVALACLGGRPALDAVKKGLPHAPEFIRRVNRRIAERTSHRVADYAHVVRVLEFFQCHSHPAHAFDEAMTQFGMSRHGLVQLFRRVGVTEFEARYGTLPPASQRWDRILQASGMKRAKPSPTSAQTPDQTSLHAFADSLERDLDAPSPMHEGDQTRASSRKRSRSDRAVTGPSAQQAVEVRVPEQRDALHLPLSWRVKRPRTRIWGGLPDPISRSQLVKSELEEKKSELRHKLKYVPHEYIELIEIARNSTQDRILEMKVMEFFMKVYGYRGKHLGGSRKPDGAIYTVGSPIDYGVIVDTKAYSGGYNLPIGQADEMQRYVEENQTRNKHINPNEWWKVYPSSVTEFKFLFVSGHFKGNYKAQLTRLNHITNCNGAVLSVEELLIGGEMIKAGTLTLEEVRRKFNNGEINF

SEQ ID NO: 37 - protein, 1137 aa, Artificial Sequence
  synthetic
MASSPPKKKRKVSWKDASGWSRMHADPIRPRRPSPARELLPGPQPDRVQPTADRGVSAPAGSPLDGLPARRTVSRTRLPSPPAPSPAFSAGSFSDLLRPFDPSLLDTSLLDSMPAVGTPHTAAAPAEWDEAQSALRAADDPPPTVRVAVTAARPPRAKPAPRRRAAQPSDASPAAQVDLRTLGYSQQQQEKIKPKVRSTVAQHHEALVGHGFTHAHIVALSQHPAALGTVAVTYQHIITALPEATHEDIVGVGKQWSGARALEALLTDAGELRGPPLQLDTGQLVKIAKRGGVTAMEAVHASRNALTGAPLNLTPAQVVAIASNIGGKQALETVQRLLPVLCQDHGLTPDQVVAIASNGGGKQALETVQRLLPVLCQDHGLTPDQVVAIASHDGGKQALETVQRLLPVLCQDHGLTPDQVVAIASNIGGKQALETVQRLLPVLCQDHGLTPDQVVAIASNIGGKQALETVQRLLPVLCQDHGLTPDQVVAIANNNGGKQALETVQRLLPVLCQDHGLTPDQVVAIASNIGGKQALETVQRLLPVLCQDHGLTPDQVVAIASNGGGKQALETVQRLLPVLCQDHGLTPDQVVAIASNGGGKQALETVQRLLPVLCQDHGLTPDQVVAIASHDGGKQALETVQRLLPVLCQDHGLTPDQVVAIASNGGGKQALETVQRLLPVLCQDHGLTPDQVVAIASHDGGKQALESIVAQLSRRDPALAALTNDHLVALACLGGRPALDAVKKGLPHAPEFIRRVNRRIAERTSHRVADYAHVVRVLEFFQCHSHPAHAFDEAMTQFGMSRHGLVQLFRRVGVTEFEARYGTLPPASQRWDRILQASGMKRAKPSPTSAQTPDQTSLHAFADSLERDLDAPSPMHEGDQTRASSRKRSRSDRAVTGPSAQQAVEVRVPEQRDALHLPLSWRVKRPRTRIWGGLPDPISRSQLVKSELEEKKSELRHKLKYVPHEYIELIEIARNSTQDRILEMKVMEFFMKVYGYRGKHLGGSRKPDGAIYTVGSPIDYGVIVDTKAYSGGYNLPIGQADEMQRYVEENQTRNKHINPNEWWKVYPSSVTEFKFLFVSGHFKGNYKAQLTRLNHITNCNGAVLSVEELLIGGEMIKAGTLTLEEVRRKFNNGEINF

SEQ ID NO: 38 - protein, 1137 aa, Artificial Sequence
  synthetic
MASSPPKKKRKVSWKDASGWSRMHADPIRPRRPSPARELLPGPQPDRVQPTADRGVSAPAGSPLDGLPARRTVSRTRLPSPPAPSPAFSAGSFSDLLRPFDPSLLDTSLLDSMPAVGTPHTAAAPAEWDEAQSALRAADDPPPTVRVAVTAARPPRAKPAPRRRAAQPSDASPAAQVDLRTLGYSQQQQEKIKPKVRSTVAQHHEALVGHGFTHAHIVALSQHPAALGTVAVTYQHIITALPEATHEDIVGVGKQWSGARALEALLTDAGELRGPPLQLDTGQLVKIAKRGGVTAMEAVHASRNALTGAPLNLTPAQVVAIASHDGGKQALETVQRLLPVLCQDHGLTPDQVVAIASHDGGKQALETVQRLLPVLCQDHGLTPDQVVAIASHDGGKQALETVQRLLPVLCQDHGLTPDQVVAIASNIGGKQALETVQRLLPVLCQDHGLTPDQVVAIANNNGGKQALETVQRLLPVLCQDHGLTPDQVVAIASNIGGKQALETVQRLLPVLCQDHGLTPDQVVAIASNIGGKQALETVQRLLPVLCQDHGLTPDQVVAIANNNGGKQALETVQRLLPVLCQDHGLTPDQVVAIASNGGGKQALETVQRLLPVLCQDHGLTPDQVVAIASNIGGKQALETVQRLLPVLCQDHGLTPDQVVAIASNIGGKQALETVQRLLPVLCQDHGLTPDQVVAIASNIGGKQALESIVAQLSRRDPALAALTNDHLVALACLGGRPALDAVKKGLPHAPEFIRRVNRRIAERTSHRVADYAHVVRVLEFFQCHSHPAHAFDEAMTQFGMSRHGLVQLFRRVGVTEFEARYGTLPPASQRWDRILQASGMKRAKPSPTSAQTPDQTSLHAFADSLERDLDAPSPMHEGDQTRASSRKRSRSDRAVTGPSAQQAVEVRVPEQRDALHLPLSWRVKRPRTRIWGGLPDPISRSQLVKSELEEKKSELRHKLKYVPHEYIELIEIARNSTQDRILEMKVMEFFMKVYGYRGKHLGGSRKPDGAIYTVGSPIDYGVIVDTKAYSGGYNLPIGQADEMQRYVEENQTRNKHINPNEWWKVYPSSVTEFKFLFVSGHFKGNYKAQLTRLNHITNCNGAVLSVEELLIGGEMIKAGTLTLEEVRRKFNNGEINF

SEQ ID NO: 39 - protein, 1137 aa, Artificial Sequence
  synthetic
MASSPPKKKRKVSWKDASGWSRMHADPIRPRRPSPARELLPGPQPDRVQPTADRGVSAPAGSPLDGLPARRTVSRTRLPSPPAPSPAFSAGSFSDLLRPFDPSLLDTSLLDSMPAVGTPHTAAAPAEWDEAQSALRAADDPPPTVRVAVTAARPPRAKPAPRRRAAQPSDASPAAQVDLRTLGYSQQQQEKIKPKVRSTVAQHHEALVGHGFTHAHIVALSQHPAALGTVAVTYQHIITALPEATHEDIVGVGKQWSGARALEALLTDAGELRGPPLQLDTGQLVKIAKRGGVTAMEAVHASRNALTGAPLNLTPAQVVAIASHDGGKQALETVQRLLPVLCQDHGLTPDQVVAIASHDGGKQALETVQRLLPVLCQDHGLTPDQVVAIANNNGGKQALETVQRLLPVLCQDHGLTPDQVVAIANNNGGKQALETVQRLLPVLCQDHGLTPDQVVAIASNIGGKQALETVQRLLPVLCQDHGLTPDQVVAIASNGGGKQALETVQRLLPVLCQDHGLTPDQVVAIANNNGGKQALETVQRLLPVLCQDHGLTPDQVVAIASHDGGKQALETVQRLLPVLCQDHGLTPDQVVAIASNGGGKQALETVQRLLPVLCQDHGLTPDQVVAIASHDGGKQALETVQRLLPVLCQDHGLTPDQVVAIASHDGGKQALETVQRLLPVLCQDHGLTPDQVVAIASNGGGKQALESIVAQLSRRDPALAALTNDHLVALACLGGRPALDAVKKGLPHAPEFIRRVNRRIAERTSHRVADYAHVVRVLEFFQCHSHPAHAFDEAMTQFGMSRHGLVQLFRRVGVTEFEARYGTLPPASQRWDRILQASGMKRAKPSPTSAQTPDQTSLHAFADSLERDLDAPSPMHEGDQTRASSRKRSRSDRAVTGPSAQQAVEVRVPEQRDALHLPLSWRVKRPRTRIWGGLPDPISRSQLVKSELEEKKSELRHKLKYVPHEYIELIEIARNSTQDRILEMKVMEFFMKVYGYRGKHLGGSRKPDGAIYTVGSPIDYGVIVDTKAYSGGYNLPIGQADEMQRYVEENQTRNKHINPNEWWKVYPSSVTEFKFLFVSGHFKGNYKAQLTRLNHITNCNGAVLSVEELLIGGEMIKAGTLTLEEVRRKFNNGEINF

SEQ ID NO: 40 - protein, 1137 aa, Artificial Sequence
  synthetic
MASSPPKKKRKVSWKDASGWSRMHADPIRPRRPSPARELLPGPQPDRVQPTADRGVSAPAGSPLDGLPARRTVSRTRLPSPPAPSPAFSAGSFSDLLRPFDPSLLDTSLLDSMPAVGTPHTAAAPAEWDEAQSALRAADDPPPTVRVAVTAARPPRAKPAPRRRAAQPSDASPAAQVDLRTLGYSQQQQEKIKPKVRSTVAQHHEALVGHGFTHAHIVALSQHPAALGTVAVTYQHIITALPEATHEDIVGVGKQWSGARALEALLTDAGELRGPPLQLDTGQLVKIAKRGGVTAMEAVHASRNALTGAPLNLTPAQVVAIASNIGGKQALETVQRLLPVLCQDHGLTPDQVVAIANNNGGKQALETVQRLLPVLCQDHGLTPDQVVAIASNIGGKQALETVQRLLPVLCQDHGLTPDQVVAIASHDGGKQALETVQRLLPVLCQDHGLTPDQVVAIASNIGGKQALETVQRLLPVLCQDHGLTPDQVVAIASNIGGKQALETVQRLLPVLCQDHGLTPDQVVAIASNIGGKQALETVQRLLPVLCQDHGLTPDQVVAIASHDGGKQALETVQRLLPVLCQDHGLTPDQVVAIASHDGGKQALETVQRLLPVLCQDHGLTPDQVVAIASNIGGKQALETVQRLLPVLCQDHGLTPDQVVAIASHDGGKQALETVQRLLPVLCQDHGLTPDQVVAIASNIGGKQALESIVAQLSRRDPALAALTNDHLVALACLGGRPALDAVKKGLPHAPEFIRRVNRRIAERTSHRVADYAHVVRVLEFFQCHSHPAHAFDEAMTQFGMSRHGLVQLFRRVGVTEFEARYGTLPPASQRWDRILQASGMKRAKPSPTSAQTPDQTSLHAFADSLERDLDAPSPMHEGDQTRASSRKRSRSDRAVTGPSAQQAVEVRVPEQRDALHLPLSWRVKRPRTRIWGGLPDPISRSQLVKSELEEKKSELRHKLKYVPHEYIELIEIARNSTQDRILEMKVMEFFMKVYGYRGKHLGGSRKPDGAIYTVGSPIDYGVIVDTKAYSGGYNLPIGQADEMQRYVEENQTRNKHINPNEWWKVYPSSVTEFKFLFVSGHFKGNYKAQLTRLNHITNCNGAVLSVEELLIGGEMIKAGTLTLEEVRRKFNNGEINF

SEQ ID NO: 41 - protein, 1137 aa, Artificial Sequence
  synthetic
MASSPPKKKRKVSWKDASGWSRMHADPIRPRRPSPARELLPGPQPDRVQPTADRGVSAPAGSPLDGLPARRTVSRTRLPSPPAPSPAFSAGSFSDLLRPFDPSLLDTSLLDSMPAVGTPHTAAAPAEWDEAQSALRAADDPPPTVRVAVTAARPPRAKPAPRRRAAQPSDASPAAQVDLRTLGYSQQQQEKIKPKVRSTVAQHHEALVGHGFTHAHIVALSQHPAALGTVAVTYQHIITALPEATHEDIVGVGKQWSGARALEALLTDAGELRGPPLQLDTGQLVKIAKRGGVTAMEAVHASRNALTGAPLNLTPAQVVAIANNNGGKQALETVQRLLPVLCQDHGLTPDQVVAIANNNGGKQALETVQRLLPVLCQDHGLTPDQVVAIASHDGGKQALETVQRLLPVLCQDHGLTPDQVVAIASNIGGKQALETVQRLLPVLCQDHGLTPDQVVAIASHDGGKQALETVQRLLPVLCQDHGLTPDQVVAIASNGGGKQALETVQRLLPVLCQDHGLTPDQVVAIANNNGGKQALETVQRLLPVLCQDHGLTPDQVVAIASHDGGKQALETVQRLLPVLCQDHGLTPDQVVAIASNGGGKQALETVQRLLPVLCQDHGLTPDQVVAIASNIGGKQALETVQRLLPVLCQDHGLTPDQVVAIASNIGGKQALETVQRLLPVLCQDHGLTPDQVVAIASHDGGKQALESIVAQLSRRDPALAALTNDHLVALACLGGRPALDAVKKGLPHAPEFIRRVNRRIAERTSHRVADYAHVVRVLEFFQCHSHPAHAFDEAMTQFGMSRHGLVQLFRRVGVTEFEARYGTLPPASQRWDRILQASGMKRAKPSPTSAQTPDQTSLHAFADSLERDLDAPSPMHEGDQTRASSRKRSRSDRAVTGPSAQQAVEVRVPEQRDALHLPLSWRVKRPRTRIWGGLPDPISRSQLVKSELEEKKSELRHKLKYVPHEYIELIEIARNSTQDRILEMKVMEFFMKVYGYRGKHLGGSRKPDGAIYTVGSPIDYGVIVDTKAYSGGYNLPIGQADEMQRYVEENQTRNKHINPNEWWKVYPSSVTEFKFLFVSGHFKGNYKAQLTRLNHITNCNGAVLSVEELLIGGEMIKAGTLTLEEVRRKFNNGEINF

SEQ ID NO: 42 - protein, 1171 aa, Artificial Sequence
  synthetic
MASSPPKKKRKVSWKDASGWSRMHADPIRPRRPSPARELLPGPQPDRVQPTADRGVSAPAGSPLDGLPARRTVSRTRLPSPPAPSPAFSAGSFSDLLRPFDPSLLDTSLLDSMPAVGTPHTAAAPAEWDEAQSALRAADDPPPTVRVAVTAARPPRAKPAPRRRAAQPSDASPAAQVDLRTLGYSQQQQEKIKPKVRSTVAQHHEALVGHGFTHAHIVALSQHPAALGTVAVTYQHIITALPEATHEDIVGVGKQWSGARALEALLTDAGELRGPPLQLDTGQLVKIAKRGGVTAMEAVHASRNALTGAPLNLTPAQVVAIASNIGGKQALETVQRLLPVLCQDHGLTPDQVVAIASHDGGKQALETVQRLLPVLCQDHGLTPDQVVAIASHDGGKQALETVQRLLPVLCQDHGLTPDQVVAIASHDGGKQALETVQRLLPVLCQDHGLTPDQVVAIASHDGGKQALETVQRLLPVLCQDHGLTPDQVVAIASNGGGKQALETVQRLLPVLCQDHGLTPDQVVAIASHDGGKQALETVQRLLPVLCQDHGLTPDQVVAIASNGGGKQALETVQRLLPVLCQDHGLTPDQVVAIASHDGGKQALETVQRLLPVLCQDHGLTPDQVVAIASHDGGKQALETVQRLLPVLCQDHGLTPDQVVAIANNNGGKQALETVQRLLPVLCQDHGLTPDQVVAIASHDGGKQALETVQRLLPVLCQDHGLTPDQVVAIASNGGGKQALESIVAQLSRRDPALAALTNDHLVALACLGGRPALDAVKKGLPHAPEFIRRVNRRIAERTSHRVADYAHVVRVLEFFQCHSHPAHAFDEAMTQFGMSRHGLVQLFRRVGVTEFEARYGTLPPASQRWDRILQASGMKRAKPSPTSAQTPDQTSLHAFADSLERDLDAPSPMHEGDQTRASSRKRSRSDRAVTGPSAQQAVEVRVPEQRDALHLPLSWRVKRPRTRIWGGLPDPISRSQLVKSELEEKKSELRHKLKYVPHEYIELIEIARNSTQDRILEMKVMEFFMKVYGYRGKHLGGSRKPDGAIYTVGSPIDYGVIVDTKAYSGGYNLPIGQADEMQRYVEENQTRNKHINPNEWWKVYPSSVTEFKFLFVSGHFKGNYKAQLTRLNHITNCNGAVLSVEELLIGGEMIKAGTLTLEEVRRKFNNGEINF

SEQ ID NO: 43 - protein, 1239 aa, Artificial Sequence
  synthetic
MASSPPKKKRKVSWKDASGWSRMHADPIRPRRPSPARELLPGPQPDRVQPTADRGVSAPAGSPLDGLPARRTVSRTRLPSPPAPSPAFSAGSFSDLLRPFDPSLLDTSLLDSMPAVGTPHTAAAPAEWDEAQSALRAADDPPPTVRVAVTAARPPRAKPAPRRRAAQPSDASPAAQVDLRTLGYSQQQQEKIKPKVRSTVAQHHEALVGHGFTHAHIVALSQHPAALGTVAVTYQHIITALPEATHEDIVGVGKQWSGARALEALLTDAGELRGPPLQLDTGQLVKIAKRGGVTAMEAVHASRNALTGAPLNLTPAQVVAIASHDGGKQALETVQRLLPVLCQDHGLTPDQVVAIASHDGGKQALETVQRLLPVLCQDHGLTPDQVVAIASHDGGKQALETVQRLLPVLCQDHGLTPDQVVAIASNIGGKQALETVQRLLPVLCQDHGLTPDQVVAIANNNGGKQALETVQRLLPVLCQDHGLTPDQVVAIASNIGGKQALETVQRLLPVLCQDHGLTPDQVVAIASNIGGKQALETVQRLLPVLCQDHGLTPDQVVAIANNNGGKQALETVQRLLPVLCQDHGLTPDQVVAIASNGGGKQALETVQRLLPVLCQDHGLTPDQVVAIASNIGGKQALETVQRLLPVLCQDHGLTPDQVVAIASNIGGKQALETVQRLLPVLCQDHGLTPDQVVAIASNIGGKQALETVQRLLPVLCQDHGLTPDQVVAIASHDGGKQALETVQRLLPVLCQDHGLTPDQVVAIASNIGGKQALETVQRLLPVLCQDHGLTPDQVVAIASNGGGKQALESIVAQLSRRDPALAALTNDHLVALACLGGRPALDAVKKGLPHAPEFIRRVNRRIAERTSHRVADYAHVVRVLEFFQCHSHPAHAFDEAMTQFGMSRHGLVQLFRRVGVTEFEARYGTLPPASQRWDRILQASGMKRAKPSPTSAQTPDQTSLHAFADSLERDLDAPSPMHEGDQTRASSRKRSRSDRAVTGPSAQQAVEVRVPEQRDALHLPLSWRVKRPRTRIWGGLPDPISRSQLVKSELEEKKSELRHKLKYVPHEYIELIEIARNSTQDRILEMKVMEFFMKVYGYRGKHLGGSRKPDGAIYTVGSPIDYGVIVDTKAYSGGYNLPIGQADEMQRYVEENQTRNKHINPNEWWKVYPSSVTEFKFLFVSGHFKGNYKAQLTRLNHITNCNGAVLSVEELLIGGEMIKAGTLTLEEVRRKFNNGEINF

SEQ ID NO: 44 - protein, 1239 aa, Artificial Sequence
  synthetic
MASSPPKKKRKVSWKDASGWSRMHADPIRPRRPSPARELLPGPQPDRVQPTADRGVSAPAGSPLDGLPARRTVSRTRLPSPPAPSPAFSAGSFSDLLRPFDPSLLDTSLLDSMPAVGTPHTAAAPAEWDEAQSALRAADDPPPTVRVAVTAARPPRAKPAPRRRAAQPSDASPAAQVDLRTLGYSQQQQEKIKPKVRSTVAQHHEALVGHGFTHAHIVALSQHPAALGTVAVTYQHIITALPEATHEDIVGVGKQWSGARALEALLTDAGELRGPPLQLDTGQLVKIAKRGGVTAMEAVHASRNALTGAPLNLTPAQVVAIASHDGGKQALETVQRLLPVLCQDHGLTPDQVVAIASHDGGKQALETVQRLLPVLCQDHGLTPDQVVAIANNNGGKQALETVQRLLPVLCQDHGLTPDQVVAIANNNGGKQALETVQRLLPVLCQDHGLTPDQVVAIASNIGGKQALETVQRLLPVLCQDHGLTPDQVVAIASNGGGKQALETVQRLLPVLCQDHGLTPDQVVAIANNNGGKQALETVQRLLPVLCQDHGLTPDQVVAIASHDGGKQALETVQRLLPVLCQDHGLTPDQVVAIASNGGGKQALETVQRLLPVLCQDHGLTPDQVVAIASHDGGKQALETVQRLLPVLCQDHGLTPDQVVAIASHDGGKQALETVQRLLPVLCQDHGLTPDQVVAIASNGGGKQALETVQRLLPVLCQDHGLTPDQVVAIASHDGGKQALETVQRLLPVLCQDHGLTPDQVVAIASNGGGKQALETVQRLLPVLCQDHGLTPDQVVAIASNGGGKQALESIVAQLSRRDPALAALTNDHLVALACLGGRPALDAVKKGLPHAPEFIRRVNRRIAERTSHRVADYAHVVRVLEFFQCHSHPAHAFDEAMTQFGMSRHGLVQLFRRVGVTEFEARYGTLPPASQRWDRILQASGMKRAKPSPTSAQTPDQTSLHAFADSLERDLDAPSPMHEGDQTRASSRKRSRSDRAVTGPSAQQAVEVRVPEQRDALHLPLSWRVKRPRTRIWGGLPDPISRSQLVKSELEEKKSELRHKLKYVPHEYIELIEIARNSTQDRILEMKVMEFFMKVYGYRGKHLGGSRKPDGAIYTVGSPIDYGVIVDTKAYSGGYNLPIGQADEMQRYVEENQTRNKHINPNEWWKVYPSSVTEFKFLFVSGHFKGNYKAQLTRLNHITNCNGAVLSVEELLIGGEMIKAGTLTLEEVRRKFNNGEINF

SEQ ID NO: 45 - protein, 1239 aa, Artificial Sequence
  synthetic
MASSPPKKKRKVSWKDASGWSRMHADPIRPRRPSPARELLPGPQPDRVQPTADRGVSAPAGSPLDGLPARRTVSRTRLPSPPAPSPAFSAGSFSDLLRPFDPSLLDTSLLDSMPAVGTPHTAAAPAEWDEAQSALRAADDPPPTVRVAVTAARPPRAKPAPRRRAAQPSDASPAAQVDLRTLGYSQQQQEKIKPKVRSTVAQHHEALVGHGFTHAHIVALSQHPAALGTVAVTYQHIITALPEATHEDIVGVGKQWSGARALEALLTDAGELRGPPLQLDTGQLVKIAKRGGVTAMEAVHASRNALTGAPLNLTPAQVVAIASNIGGKQALETVQRLLPVLCQDHGLTPDQVVAIANNNGGKQALETVQRLLPVLCQDHGLTPDQVVAIASNIGGKQALETVQRLLPVLCQDHGLTPDQVVAIASHDGGKQALETVQRLLPVLCQDHGLTPDQVVAIASNIGGKQALETVQRLLPVLCQDHGLTPDQVVAIASNIGGKQALETVQRLLPVLCQDHGLTPDQVVAIASNIGGKQALETVQRLLPVLCQDHGLTPDQVVAIASHDGGKQALETVQRLLPVLCQDHGLTPDQVVAIASHDGGKQALETVQRLLPVLCQDHGLTPDQVVAIASNIGGKQALETVQRLLPVLCQDHGLTPDQVVAIASHDGGKQALETVQRLLPVLCQDHGLTPDQVVAIASNIGGKQALETVQRLLPVLCQDHGLTPDQVVAIASNIGGKQALETVQRLLPVLCQDHGLTPDQVVAIASHDGGKQALETVQRLLPVLCQDHGLTPDQVVAIASNGGGKQALESIVAQLSRRDPALAALTNDHLVALACLGGRPALDAVKKGLPHAPEFIRRVNRRIAERTSHRVADYAHVVRVLEFFQCHSHPAHAFDEAMTQFGMSRHGLVQLFRRVGVTEFEARYGTLPPASQRWDRILQASGMKRAKPSPTSAQTPDQTSLHAFADSLERDLDAPSPMHEGDQTRASSRKRSRSDRAVTGPSAQQAVEVRVPEQRDALHLPLSWRVKRPRTRIWGGLPDPISRSQLVKSELEEKKSELRHKLKYVPHEYIELIEIARNSTQDRILEMKVMEFFMKVYGYRGKHLGGSRKPDGAIYTVGSPIDYGVIVDTKAYSGGYNLPIGQADEMQRYVEENQTRNKHINPNEWWKVYPSSVTEFKFLFVSGHFKGNYKAQLTRLNHITNCNGAVLSVEELLIGGEMIKAGTLTLEEVRRKFNNGEINF

SEQ ID NO: 46 - protein, 1239 aa, Artificial Sequence
  synthetic
MASSPPKKKRKVSWKDASGWSRMHADPIRPRRPSPARELLPGPQPDRVQPTADRGVSAPAGSPLDGLPARRTVSRTRLPSPPAPSPAFSAGSFSDLLRPFDPSLLDTSLLDSMPAVGTPHTAAAPAEWDEAQSALRAADDPPPTVRVAVTAARPPRAKPAPRRRAAQPSDASPAAQVDLRTLGYSQQQQEKIKPKVRSTVAQHHEALVGHGFTHAHIVALSQHPAALGTVAVTYQHIITALPEATHEDIVGVGKQWSGARALEALLTDAGELRGPPLQLDTGQLVKIAKRGGVTAMEAVHASRNALTGAPLNLTPAQVVAIANNNGGKQALETVQRLLPVLCQDHGLTPDQVVAIANNNGGKQALETVQRLLPVLCQDHGLTPDQVVAIASHDGGKQALETVQRLLPVLCQDHGLTPDQVVAIASNIGGKQALETVQRLLPVLCQDHGLTPDQVVAIASHDGGKQALETVQRLLPVLCQDHGLTPDQVVAIASNGGGKQALETVQRLLPVLCQDHGLTPDQVVAIANNNGGKQALETVQRLLPVLCQDHGLTPDQVVAIASHDGGKQALETVQRLLPVLCQDHGLTPDQVVAIASNGGGKQALETVQRLLPVLCQDHGLTPDQVVAIASNIGGKQALETVQRLLPVLCQDHGLTPDQVVAIASNIGGKQALETVQRLLPVLCQDHGLTPDQVVAIASHDGGKQALETVQRLLPVLCQDHGLTPDQVVAIASHDGGKQALETVQRLLPVLCQDHGLTPDQVVAIASHDGGKQALETVQRLLPVLCQDHGLTPDQVVAIASNGGGKQALESIVAQLSRRDPALAALTNDHLVALACLGGRPALDAVKKGLPHAPEFIRRVNRRIAERTSHRVADYAHVVRVLEFFQCHSHPAHAFDEAMTQFGMSRHGLVQLFRRVGVTEFEARYGTLPPASQRWDRILQASGMKRAKPSPTSAQTPDQTSLHAFADSLERDLDAPSPMHEGDQTRASSRKRSRSDRAVTGPSAQQAVEVRVPEQRDALHLPLSWRVKRPRTRIWGGLPDPISRSQLVKSELEEKKSELRHKLKYVPHEYIELIEIARNSTQDRILEMKVMEFFMKVYGYRGKHLGGSRKPDGAIYTVGSPIDYGVIVDTKAYSGGYNLPIGQADEMQRYVEENQTRNKHINPNEWWKVYPSSVTEFKFLFVSGHFKGNYKAQLTRLNHITNCNGAVLSVEELLIGGEMIKAGTLTLEEVRRKFNNGEINF

SEQ ID NO: 47 - protein, 1239 aa, Artificial Sequence
  synthetic
MASSPPKKKRKVSWKDASGWSRMHADPIRPRRPSPARELLPGPQPDRVQPTADRGVSAPAGSPLDGLPARRTVSRTRLPSPPAPSPAFSAGSFSDLLRPFDPSLLDTSLLDSMPAVGTPHTAAAPAEWDEAQSALRAADDPPPTVRVAVTAARPPRAKPAPRRRAAQPSDASPAAQVDLRTLGYSQQQQEKIKPKVRSTVAQHHEALVGHGFTHAHIVALSQHPAALGTVAVTYQHIITALPEATHEDIVGVGKQWSGARALEALLTDAGELRGPPLQLDTGQLVKIAKRGGVTAMEAVHASRNALTGAPLNLTPAQVVAIASHDGGKQALETVQRLLPVLCQDHGLTPDQVVAIASNGGGKQALETVQRLLPVLCQDHGLTPDQVVAIASNGGGKQALETVQRLLPVLCQDHGLTPDQVVAIANNNGGKQALETVQRLLPVLCQDHGLTPDQVVAIASNGGGKQALETVQRLLPVLCQDHGLTPDQVVAIASHDGGKQALETVQRLLPVLCQDHGLTPDQVVAIASHDGGKQALETVQRLLPVLCQDHGLTPDQVVAIANNNGGKQALETVQRLLPVLCQDHGLTPDQVVAIASHDGGKQALETVQRLLPVLCQDHGLTPDQVVAIASNIGGKQALETVQRLLPVLCQDHGLTPDQVVAIASNGGGKQALETVQRLLPVLCQDHGLTPDQVVAIANNNGGKQALETVQRLLPVLCQDHGLTPDQVVAIASNIGGKQALETVQRLLPVLCQDHGLTPDQVVAIASNGGGKQALETVQRLLPVLCQDHGLTPDQVVAIASNGGGKQALESIVAQLSRRDPALAALTNDHLVALACLGGRPALDAVKKGLPHAPEFIRRVNRRIAERTSHRVADYAHVVRVLEFFQCHSHPAHAFDEAMTQFGMSRHGLVQLFRRVGVTEFEARYGTLPPASQRWDRILQASGMKRAKPSPTSAQTPDQTSLHAFADSLERDLDAPSPMHEGDQTRASSRKRSRSDRAVTGPSAQQAVEVRVPEQRDALHLPLSWRVKRPRTRIWGGLPDPISRSQLVKSELEEKKSELRHKLKYVPHEYIELIEIARNSTQDRILEMKVMEFFMKVYGYRGKHLGGSRKPDGAIYTVGSPIDYGVIVDTKAYSGGYNLPIGQADEMQRYVEENQTRNKHINPNEWWKVYPSSVTEFKFLFVSGHFKGNYKAQLTRLNHITNCNGAVLSVEELLIGGEMIKAGTLTLEEVRRKFNNGEINF

SEQ ID NO: 48 - protein, 1239 aa, Artificial Sequence
  synthetic
MASSPPKKKRKVSWKDASGWSRMHADPIRPRRPSPARELLPGPQPDRVQPTADRGVSAPAGSPLDGLPARRTVSRTRLPSPPAPSPAFSAGSFSDLLRPFDPSLLDTSLLDSMPAVGTPHTAAAPAEWDEAQSALRAADDPPPTVRVAVTAARPPRAKPAPRRRAAQPSDASPAAQVDLRTLGYSQQQQEKIKPKVRSTVAQHHEALVGHGFTHAHIVALSQHPAALGTVAVTYQHIITALPEATHEDIVGVGKQWSGARALEALLTDAGELRGPPLQLDTGQLVKIAKRGGVTAMEAVHASRNALTGAPLNLTPAQVVAIASHDGGKQALETVQRLLPVLCQDHGLTPDQVVAIANNNGGKQALETVQRLLPVLCQDHGLTPDQVVAIANNNGGKQALETVQRLLPVLCQDHGLTPDQVVAIASNGGGKQALETVQRLLPVLCQDHGLTPDQVVAIASNGGGKQALETVQRLLPVLCQDHGLTPDQVVAIASNGGGKQALETVQRLLPVLCQDHGLTPDQVVAIANNNGGKQALETVQRLLPVLCQDHGLTPDQVVAIASHDGGKQALETVQRLLPVLCQDHGLTPDQVVAIASNGGGKQALETVQRLLPVLCQDHGLTPDQVVAIASNIGGKQALETVQRLLPVLCQDHGLTPDQVVAIASNGGGKQALETVQRLLPVLCQDHGLTPDQVVAIASHDGGKQALETVQRLLPVLCQDHGLTPDQVVAIANNNGGKQALETVQRLLPVLCQDHGLTPDQVVAIASNGGGKQALETVQRLLPVLCQDHGLTPDQVVAIASNGGGKQALESIVAQLSRRDPALAALTNDHLVALACLGGRPALDAVKKGLPHAPEFIRRVNRRIAERTSHRVADYAHVVRVLEFFQCHSHPAHAFDEAMTQFGMSRHGLVQLFRRVGVTEFEARYGTLPPASQRWDRILQASGMKRAKPSPTSAQTPDQTSLHAFADSLERDLDAPSPMHEGDQTRASSRKRSRSDRAVTGPSAQQAVEVRVPEQRDALHLPLSWRVKRPRTRIWGGLPDPISRSQLVKSELEEKKSELRHKLKYVPHEYIELIEIARNSTQDRILEMKVMEFFMKVYGYRGKHLGGSRKPDGAIYTVGSPIDYGVIVDTKAYSGGYNLPIGQADEMQRYVEENQTRNKHINPNEWWKVYPSSVTEFKFLFVSGHFKGNYKAQLTRLNHITNCNGAVLSVEELLIGGEMIKAGTLTLEEVRRKFNNGEINF

SEQ ID NO: 49 - protein, 1273 aa, Artificial Sequence
  synthetic
MASSPPKKKRKVSWKDASGWSRMHADPIRPRRPSPARELLPGPQPDRVQPTADRGVSAPAGSPLDGLPARRTVSRTRLPSPPAPSPAFSAGSFSDLLRPFDPSLLDTSLLDSMPAVGTPHTAAAPAEWDEAQSALRAADDPPPTVRVAVTAARPPRAKPAPRRRAAQPSDASPAAQVDLRTLGYSQQQQEKIKPKVRSTVAQHHEALVGHGFTHAHIVALSQHPAALGTVAVTYQHIITALPEATHEDIVGVGKQWSGARALEALLTDAGELRGPPLQLDTGQLVKIAKRGGVTAMEAVHASRNALTGAPLNLTPAQVVAIASNIGGKQALETVQRLLPVLCQDHGLTPDQVVAIASHDGGKQALETVQRLLPVLCQDHGLTPDQVVAIASHDGGKQALETVQRLLPVLCQDHGLTPDQVVAIASHDGGKQALETVQRLLPVLCQDHGLTPDQVVAIASHDGGKQALETVQRLLPVLCQDHGLTPDQVVAIASNGGGKQALETVQRLLPVLCQDHGLTPDQVVAIASHDGGKQALETVQRLLPVLCQDHGLTPDQVVAIASNGGGKQALETVQRLLPVLCQDHGLTPDQVVAIASHDGGKQALETVQRLLPVLCQDHGLTPDQVVAIASHDGGKQALETVQRLLPVLCQDHGLTPDQVVAIANNNGGKQALETVQRLLPVLCQDHGLTPDQVVAIASHDGGKQALETVQRLLPVLCQDHGLTPDQVVAIASNGGGKQALETVQRLLPVLCQDHGLTPDQVVAIASNGGGKQALETVQRLLPVLCQDHGLTPDQVVAIASHDGGKQALETVQRLLPVLCQDHGLTPDQVVAIASNGGGKQALESIVAQLSRRDPALAALTNDHLVALACLGGRPALDAVKKGLPHAPEFIRRVNRRIAERTSHRVADYAHVVRVLEFFQCHSHPAHAFDEAMTQFGMSRHGLVQLFRRVGVTEFEARYGTLPPASQRWDRILQASGMKRAKPSPTSAQTPDQTSLHAFADSLERDLDAPSPMHEGDQTRASSRKRSRSDRAVTGPSAQQAVEVRVPEQRDALHLPLSWRVKRPRTRIWGGLPDPISRSQLVKSELEEKKSELRHKLKYVPHEYIELIEIARNSTQDRILEMKVMEFFMKVYGYRGKHLGGSRKPDGAIYTVGSPIDYGVIVDTKAYSGGYNLPIGQADEMQRYVEENQTRNKHINPNEWWKVYPSSVTEFKFLFVSGHFKGNYKAQLTRLNHITNCNGAVLSVEELLIGGEMIKAGTLTLEEVRRKFNNGEINF

SEQ ID NO: 50 - protein, 1273 aa, Artificial Sequence
  synthetic
MASSPPKKKRKVSWKDASGWSRMHADPIRPRRPSPARELLPGPQPDRVQPTADRGVSAPAGSPLDGLPARRTVSRTRLPSPPAPSPAFSAGSFSDLLRPFDPSLLDTSLLDSMPAVGTPHTAAAPAEWDEAQSALRAADDPPPTVRVAVTAARPPRAKPAPRRRAAQPSDASPAAQVDLRTLGYSQQQQEKIKPKVRSTVAQHHEALVGHGFTHAHIVALSQHPAALGTVAVTYQHIITALPEATHEDIVGVGKQWSGARALEALLTDAGELRGPPLQLDTGQLVKIAKRGGVTAMEAVHASRNALTGAPLNLTPAQVVAIASHDGGKQALETVQRLLPVLCQDHGLTPDQVVAIASHDGGKQALETVQRLLPVLCQDHGLTPDQVVAIASHDGGKQALETVQRLLPVLCQDHGLTPDQVVAIASNNGGKQALETVQRLLPVLCQDHGLTPDQVVAIASNNGGKQALETVQRLLPVLCQDHGLTPDQVVAIASNIGGKQALETVQRLLPVLCQDHGLTPDQVVAIASNIGGKQALETVQRLLPVLCQDHGLTPDQVVAIASNNGGKQALETVQRLLPVLCQDHGLTPDQVVAIASHDGGKQALETVQRLLPVLCQDHGLTPDQVVAIASHDGGKQALETVQRLLPVLCQDHGLTPDQVVAIASNNGGKQALETVQRLLPVLCQDHGLTPDQVVAIASNIGGKQALETVQRLLPVLCQDHGLTPDQVVAIASNGGGKQALETVQRLLPVLCQDHGLTPDQVVAIASNNGGKQALETVQRLLPVLCQDHGLTPDQVVAIASHDGGKQALETVQRLLPVLCQDHGLTPDQVVAIASNGGGKQALESIVAQLSRPDPALAALTNDHLVALACLGGRPAMDAVKKGLPHAPELIRRVNRRIGERTSHRVADYAQVVRVLEFFQCHSHPAYAFDEAMTQFGMSRNGLVQLFRRVGVTELEARGGTLPPASQRWDRILQASGMKRAKPSPTSAQTPDQASLHAFADSLERDLDAPSPMHEGDQTRASSRKRSRSDRAVTGPSAQQAVEVRVPEQRDALHLPLSWRVKRPRTRIWGGLPDPISRSQLVKSELEEKKSELRHKLKYVPHEYIELIEIARNSTQDRILEMKVMEFFMKVYGYRGKHLGGSRKPDGAIYTVGSPIDYGVIVDTKAYSGGYNLPIGQADEMQRYVEENQTRNKHINPNEWWKVYPSSVTEFKFLFVSGHFKGNYKAQLTRLNHITNCNGAVLSVEELLIGGEMIKAGTLTLEEVRRKFNNGEINF

SEQ ID NO: 51 - protein, 1273 aa, Artificial Sequence
  synthetic
MASSPPKKKRKVSWKDASGWSRMHADPIRPRRPSPARELLPGPQPDRVQPTADRGVSAPAGSPLDGLPARRTVSRTRLPSPPAPSPAFSAGSFSDLLRPFDPSLLDTSLLDSMPAVGTPHTAAAPAEWDEAQSALRAADDPPPTVRVAVTAARPPRAKPAPRRRAAQPSDASPAAQVDLRTLGYSQQQQEKIKPKVRSTVAQHHEALVGHGFTHAHIVALSQHPAALGTVAVTYQHIITALPEATHEDIVGVGKQWSGARALEALLTDAGELRGPPLQLDTGQLVKIAKRGGVTAMEAVHASRNALTGAPLNLTPAQVVAIASNIGGKQALETVQRLLPVLCQDHGLTPDQVVAIASNGGGKQALETVQRLLPVLCQDHGLTPDQVVAIASNGGGKQALETVQRLLPVLCQDHGLTPDQVVAIASHDGGKQALETVQRLLPVLCQDHGLTPDQVVAIASHDGGKQALETVQRLLPVLCQDHGLTPDQVVAIASHDGGKQALETVQRLLPVLCQDHGLTPDQVVAIASHDGGKQALETVQRLLPVLCQDHGLTPDQVVAIASNIGGKQALETVQRLLPVLCQDHGLTPDQVVAIASHDGGKQALETVQRLLPVLCQDHGLTPDQVVAIANNNGGKQALETVQRLLPVLCQDHGLTPDQVVAIASNIGGKQALETVQRLLPVLCQDHGLTPDQVVAIANNNGGKQALETVQRLLPVLCQDHGLTPDQVVAIASHDGGKQALETVQRLLPVLCQDHGLTPDQVVAIASNGGGKQALETVQRLLPVLCQDHGLTPDQVVAIASHDGGKQALETVQRLLPVLCQDHGLTPDQVVAIASNGGGKQALESIVAQLSRRDPALAALTNDHLVALACLGGRPALDAVKKGLPHAPEFIRRVNRRIAERTSHRVADYAHVVRVLEFFQCHSHPAHAFDEAMTQFGMSRHGLVQLFRRVGVTEFEARYGTLPPASQRWDRILQASGMKRAKPSPTSAQTPDQTSLHAFADSLERDLDAPSPMHEGDQTRASSRKRSRSDRAVTGPSAQQAVEVRVPEQRDALHLPLSWRVKRPRTRIWGGLPDPISRSQLVKSELEEKKSELRHKLKYVPHEYIELIEIARNSTQDRILEMKVMEFFMKVYGYRGKHLGGSRKPDGAIYTVGSPIDYGVIVDTKAYSGGYNLPIGQADEMQRYVEENQTRNKHINPNEWWKVYPSSVTEFKFLFVSGHFKGNYKAQLTRLNHITNCNGAVLSVEELLIGGEMIKAGTLTLEEVRRKFNNGEINF

SEQ ID NO: 52 - protein, 1307 aa, Artificial Sequence
  synthetic
MASSPPKKKRKVSWKDASGWSRMHADPIRPRRPSPARELLPGPQPDRVQPTADRGVSAPAGSPLDGLPARRTVSRTRLPSPPAPSPAFSAGSFSDLLRPFDPSLLDTSLLDSMPAVGTPHTAAAPAEWDEAQSALRAADDPPPTVRVAVTAARPPRAKPAPRRRAAQPSDASPAAQVDLRTLGYSQQQQEKIKPKVRSTVAQHHEALVGHGFTHAHIVALSQHPAALGTVAVTYQHIITALPEATHEDIVGVGKQWSGARALEALLTDAGELRGPPLQLDTGQLVKIAKRGGVTAMEAVHASRNALTGAPLNLTPAQVVAIASNIGGKQALETVQRLLPVLCQDHGLTPDQVVAIANNNGGKQALETVQRLLPVLCQDHGLTPDQVVAIASNIGGKQALETVQRLLPVLCQDHGLTPDQVVAIASHDGGKQALETVQRLLPVLCQDHGLTPDQVVAIASNIGGKQALETVQRLLPVLCQDHGLTPDQVVAIANNNGGKQALETVQRLLPVLCQDHGLTPDQVVAIANNNGGKQALETVQRLLPVLCQDHGLTPDQVVAIASNIGGKQALETVQRLLPVLCQDHGLTPDQVVAIASNIGGKQALETVQRLLPVLCQDHGLTPDQVVAIANNNGGKQALETVQRLLPVLCQDHGLTPDQVVAIASNGGGKQALETVQRLLPVLCQDHGLTPDQVVAIANNNGGKQALETVQRLLPVLCQDHGLTPDQVVAIANNNGGKQALETVQRLLPVLCQDHGLTPDQVVAIASNIGGKQALETVQRLLPVLCQDHGLTPDQVVAIANNNGGKQALETVQRLLPVLCQDHGLTPDQVVAIASHDGGKQALETVQRLLPVLCQDHGLTPDQVVAIASNGGGKQALESIVAQLSRRDPALAALTNDHLVALACLGGRPALDAVKKGLPHAPEFIRRVNRRIAERTSHRVADYAHVVRVLEFFQCHSHPAHAFDEAMTQFGMSRHGLVQLFRRVGVTEFEARYGTLPPASQRWDRILQASGMKRAKPSPTSAQTPDQTSLHAFADSLERDLDAPSPMHEGDQTRASSRKRSRSDRAVTGPSAQQAVEVRVPEQRDALHLPLSWRVKRPRTRIWGGLPDPISRSQLVKSELEEKKSELRHKLKYVPHEYIELIEIARNSTQDRILEMKVMEFFMKVYGYRGKHLGGSRKPDGAIYTVGSPIDYGVIVDTKAYSGGYNLPIGQADEMQRYVEENQTRNKHINPNEWWKVYPSSVTEFKFLFVSGHFKGNYKAQLTRLNHITNCNGAVLSVEELLIGGEMIKAGTLTLEEVRRKFNNGEINF

SEQ ID NO: 53 - protein, 1341 aa, Artificial Sequence
  synthetic
MASSPPKKKRKVSWKDASGWSRMHADPIRPRRPSPARELLPGPQPDRVQPTADRGVSAPAGSPLDGLPARRTVSRTRLPSPPAPSPAFSAGSFSDLLRPFDPSLLDTSLLDSMPAVGTPHTAAAPAEWDEAQSALRAADDPPPTVRVAVTAARPPRAKPAPRRRAAQPSDASPAAQVDLRTLGYSQQQQEKIKPKVRSTVAQHHEALVGHGFTHAHIVALSQHPAALGTVAVTYQHIITALPEATHEDIVGVGKQWSGARALEALLTDAGELRGPPLQLDTGQLVKIAKRGGVTAMEAVHASRNALTGAPLNLTPAQVVAIASNIGGKQALETVQRLLPVLCQDHGLTPDQVVAIASNGGGKQALETVQRLLPVLCQDHGLTPDQVVAIASHDGGKQALETVQRLLPVLCQDHGLTPDQVVAIASNIGGKQALETVQRLLPVLCQDHGLTPDQVVAIASNIGGKQALETVQRLLPVLCQDHGLTPDQVVAIANNNGGKQALETVQRLLPVLCQDHGLTPDQVVAIASNIGGKQALETVQRLLPVLCQDHGLTPDQVVAIASNGGGKQALETVQRLLPVLCQDHGLTPDQVVAIASNGGGKQALETVQRLLPVLCQDHGLTPDQVVAIASHDGGKQALETVQRLLPVLCQDHGLTPDQVVAIASNGGGKQALETVQRLLPVLCQDHGLTPDQVVAIASHDGGKQALETVQRLLPVLCQDHGLTPDQVVAIASNGGGKQALETVQRLLPVLCQDHGLTPDQVVAIASNGGGKQALETVQRLLPVLCQDHGLTPDQVVAIASHDGGKQALETVQRLLPVLCQDHGLTPDQVVAIASNIGGKQALETVQRLLPVLCQDHGLTPDQVVAIASHDGGKQALETVQRLLPVLCQDHGLTPDQVVAIASNGGGKQALESIVAQLSRRDPALAALTNDHLVALACLGGRPALDAVKKGLPHAPEFIRRVNRRIAERTSHRVADYAHVVRVLEFFQCHSHPAHAFDEAMTQFGMSRHGLVQLFRRVGVTEFEARYGTLPPASQRWDRILQASGMKRAKPSPTSAQTPDQTSLHAFADSLERDLDAPSPMHEGDQTRASSRKRSRSDRAVTGPSAQQAVEVRVPEQRDALHLPLSWRVKRPRTRIWGGLPDPISRSQLVKSELEEKKSELRHKLKYVPHEYIELIEIARNSTQDRILEMKVMEFFMKVYGYRGKHLGGSRKPDGAIYTVGSPIDYGVIVDTKAYSGGYNLPIGQADEMQRYVEENQTRNKHINPNEWWKVYPSSVTEFKFLFVSGHFKGNYKAQLTRLNHITNCNGAVLSVEELLIGGEMIKAGTLTLEEVRRKFNNGEINF

SEQ ID NO: 54 - protein, 1341 aa, Artificial Sequence
  synthetic
MASSPPKKKRKVSWKDASGWSRMHADPIRPRRPSPARELLPGPQPDRVQPTADRGVSAPAGSPLDGLPARRTVSRTRLPSPPAPSPAFSAGSFSDLLRPFDPSLLDTSLLDSMPAVGTPHTAAAPAEWDEAQSALRAADDPPPTVRVAVTAARPPRAKPAPRRRAAQPSDASPAAQVDLRTLGYSQQQQEKIKPKVRSTVAQHHEALVGHGFTHAHIVALSQHPAALGTVAVTYQHIITALPEATHEDIVGVGKQWSGARALEALLTDAGELRGPPLQLDTGQLVKIAKRGGVTAMEAVHASRNALTGAPLNLTPAQVVAIASNIGGKQALETVQRLLPVLCQDHGLTPDQVVAIASHDGGKQALETVQRLLPVLCQDHGLTPDQVVAIASNGGGKQALETVQRLLPVLCQDHGLTPDQVVAIASHDGGKQALETVQRLLPVLCQDHGLTPDQVVAIASHDGGKQALETVQRLLPVLCQDHGLTPDQVVAIASNNGGKQALETVQRLLPVLCQDHGLTPDQVVAIASHDGGKQALETVQRLLPVLCQDHGLTPDQVVAIASHDGGKQALETVQRLLPVLCQDHGLTPDQVVAIASNGGGKQALETVQRLLPVLCQDHGLTPDQVVAIASNNGGKQALETVQRLLPVLCQDHGLTPDQVVAIASNIGGKQALETVQRLLPVLCQDHGLTPDQVVAIASNIGGKQALETVQRLLPVLCQDHGLTPDQVVAIASNNGGKQALETVQRLLPVLCQDHGLTPDQVVAIASHDGGKQALETVQRLLPVLCQDHGLTPDQVVAIASNIGGKQALETVQRLLPVLCQDHGLTPDQVVAIASHDGGKQALETVQRLLPVLCQDHGLTPDQVVAIASNIGGKQALETVQRLLPVLCQDHGLTPDQVVAIASNGGGKQALESIVAQLSRPDPALAALTNDHLVALACLGGRPAMDAVKKGLPHAPELIRRVNRRIGERTSHRVADYAQVVRVLEFFQCHSHPAYAFDEAMTQFGMSRNGLVQLFRRVGVTELEARGGTLPPASQRWDRILQASGMKRAKPSPTSAQTPDQASLHAFADSLERDLDAPSPMHEGDQTRASSRKRSRSDRAVTGPSAQQAVEVRVPEQRDALHLPLSWRVKRPRTRIWGGLPDPISRSQLVKSELEEKKSELRHKLKYVPHEYIELIEIARNSTQDRILEMKVMEFFMKVYGYRGKHLGGSRKPDGAIYTVGSPIDYGVIVDTKAYSGGYNLPIGQADEMQRYVEENQTRNKHINPNEWWKVYPSSVTEFKFLFVSGHFKGNYKAQLTRLNHITNCNGAVLSVEELLIGGEMIKAGTLTLEEVRRKFNNGEINF

SEQ ID NO: 55 - protein, 1341 aa, Artificial Sequence
  synthetic
MASSPPKKKRKVSWKDASGWSRMHADPIRPRRPSPARELLPGPQPDRVQPTADRGVSAPAGSPLDGLPARRTVSRTRLPSPPAPSPAFSAGSFSDLLRPFDPSLLDTSLLDSMPAVGTPHTAAAPAEWDEAQSALRAADDPPPTVRVAVTAARPPRAKPAPRRRAAQPSDASPAAQVDLRTLGYSQQQQEKIKPKVRSTVAQHHEALVGHGFTHAHIVALSQHPAALGTVAVTYQHIITALPEATHEDIVGVGKQWSGARALEALLTDAGELRGPPLQLDTGQLVKIAKRGGVTAMEAVHASRNALTGAPLNLTPAQVVAIASNNGGKQALETVQRLLPVLCQDHGLTPDQVVAIASNNGGKQALETVQRLLPVLCQDHGLTPDQVVAIASHDGGKQALETVQRLLPVLCQDHGLTPDQVVAIASNGGGKQALETVQRLLPVLCQDHGLTPDQVVAIASHDGGKQALETVQRLLPVLCQDHGLTPDQVVAIASNIGGKQALETVQRLLPVLCQDHGLTPDQVVAIASHDGGKQALETVQRLLPVLCQDHGLTPDQVVAIASHDGGKQALETVQRLLPVLCQDHGLTPDQVVAIASNGGGKQALETVQRLLPVLCQDHGLTPDQVVAIASNIGGKQALETVQRLLPVLCQDHGLTPDQVVAIASHDGGKQALETVQRLLPVLCQDHGLTPDQVVAIASNIGGKQALETVQRLLPVLCQDHGLTPDQVVAIASNIGGKQALETVQRLLPVLCQDHGLTPDQVVAIASHDGGKQALETVQRLLPVLCQDHGLTPDQVVAIASNNGGKQALETVQRLLPVLCQDHGLTPDQVVAIASNIGGKQALETVQRLLPVLCQDHGLTPDQVVAIASHDGGKQALETVQRLLPVLCQDHGLTPDQVVAIASNIGGKQALESIVAQLSRPDPALAALTNDHLVALACLGGRPAMDAVKKGLPHAPELIRRVNRRIGERTSHRVADYAQVVRVLEFFQCHSHPAYAFDEAMTQFGMSRNGLVQLFRRVGVTELEARGGTLPPASQRWDRILQASGMKRAKPSPTSAQTPDQASLHAFADSLERDLDAPSPMHEGDQTRASSRKRSRSDRAVTGPSAQQAVEVRVPEQRDALHLPLSWRVKRPRTRIWGGLPDPISRSQLVKSELEEKKSELRHKLKYVPHEYIELIEIARNSTQDRILEMKVMEFFMKVYGYRGKHLGGSRKPDGAIYTVGSPIDYGVIVDTKAYSGGYNLPIGQADEMQRYVEENQTRNKHINPNEWWKVYPSSVTEFKFLFVSGHFKGNYKAQLTRLNHITNCNGAVLSVEELLIGGEMIKAGTLTLEEVRRKFNNGEINF

SEQ ID NO: 56 - DNA, 51 bp, Arabidopsis
tatcaagattctcttcacttctctctgtcacaccgatgtttacttctggga

SEQ ID NO: 57 - DNA, 50 bp, Arabidopsis
tccggatgctcctcttgacaaggtctgtattgtcagttgtggtttgtcta

SEQ ID NO: 58 - DNA, 48 bp, Arabidopsis
ccggatgctcctcttgacaaggtctgtattgtcagttgtggtttgtct

SEQ ID NO: 59 - DNA, 40 bp, Artificial Sequence
  modified Arabidopsis
ccggatgctcctcttgacaattgtcagttgtggtttgtct

SEQ ID NO: 60 - DNA, 43 bp, Artificial Sequence
  modified Arabidopsis
ccggatgctcctcttgacaagtattgtcagttgtggtttgtct

SEQ ID NO: 61 - DNA, 33 bp, Artificial Sequence
  modified Arabidopsis
ccggatgctcctcttgacaattgtggtttgtct

SEQ ID NO: 62 - DNA, 43 bp, Artificial Sequence
  modified Arabidopsis
ccggatgctcctcttgacaaggattgtcagttgtggtttgtct

SEQ ID NO: 63 - DNA, 41 bp, Artificial Sequence
  modified Arabidopsis
ccggatgctcctcttgacaaattgtcagttgtggtttgtct

SEQ ID NO: 64 - DNA, 44 bp, Artificial Sequence
  modified Arabidopsis
ccggatgctcctcttgacaaggtattgtcagttgtggtttgtct

SEQ ID NO: 65 - protein, 34 aa, Xanthomonas gardneri
LDTGQLFKIAKRGGVTAVEAVHAWRNALTGAPLN

SEQ ID NO: 66 - protein, 34 aa, Xanthomonas campestris
LDTGQLLKIAKRGGVTAVEAVHAWRNALTGAPLN

SEQ ID NO: 67 - protein, 34 aa, Xanthomonas oryzae
LDTGQLVKIAKRGGVTAVEAVHASRNALTGAPLN

SEQ ID NO: 68 - protein, 34 aa, Xanthomonas citri; identical to SEQ ID NO: 66

SEQ ID NO: 69 - protein, 34 aa, Xanthomonas oryzae
LDTGQLVKIAKRGGVTAMEAVHASRNALTGAPLN

SEQ ID NO: 70 - protein, 34 aa, Xanthomonas oryzae; identical to SEQ ID NO: 69

SEQ ID NO: 71 - protein, 34 aa, Xanthomonas oryzae
LTPAQVVAIASNNGGKQALETVQRLLPVLCQAHG

SEQ ID NO: 72 - protein, 1307 aa, Artificial Sequence
  synthetic
MASSPPKKKRKVSWKDASGWSRMHADPIRPRRPSPARELLPGPQPDRVQPTADRGVSAPAGSPLDGLPARRTVSRTRLPSPPAPSPAFSAGSFSDLLRPFDPSLLDTSLLDSMPAVGTPHTAAAPAEWDEAQSALRAADDPPPTVRVAVTAARPPRAKPAPRRRAAQPSDASPAAQVDLRTLGYSQQQQEKIKPKVRSTVAQHHEALVGHGFTHAHIVALSQHPAALGTVAVTYQHIITALPEATHEDIVGVGKQWSGARALEALLTDAGELRGPPLQLDTGQLVKIAKRGGVTAMEAVHASRNALTGAPLNLTPAQVVAIASNNGGKQALETVQRLLPVLCQDHGLTPDQVVAIASHDGGKQALETVQRLLPVLCQDHGLTPDQVVAIASNIGGKQALETVQRLLPVLCQDHGLTPDQVVAIASNGGGKQALETVQRLLPVLCQDHGLTPDQVVAIASNIGGKQALETVQRLLPVLCQDHGLTPDQVVAIASHDGGKQALETVQRLLPVLCQDHGLTPDQVVAIASHDGGKQALETVQRLLPVLCQDHGLTPDQVVAIASNGGGKQALETVQRLLPVLCQDHGLTPDQVVAIASNIGGKQALETVQRLLPVLCQDHGLTPDQVVAIASNIGGKQALETVQRLLPVLCQDHGLTPDQVVAIASNGGGKQALETVQRLLPVLCQDHGLTPDQVVAIASHDGGKQALETVQRLLPVLCQDHGLTPDQVVAIASNIGGKQALETVQRLLPVLCQDHGLTPDQVVAIASNGGGKQALETVQRLLPVLCQDHGLTPDQVVAIASNGGGKQALETVQRLLPVLCQDHGLTPDQVVAIASNIGGKQALETVQRLLPVLCQDHGLTPDQVVAIASNGGGKQALESIVAQLSRPDPALAALTNDHLVALACLGGRPAMDAVKKGLPHAPELIRRVNRRIGERTSHRVADYAQVVRVLEFFQCHSHPAYAFDEAMTQFGMSRNGLVQLFRRVGVTELEARGGTLPPASQRWDRILQASGMKRAKPSPTSAQTPDQASLHAFADSLERDLDAPSPMHEGDQTRASSRKRSRSDRAVTGPSAQQAVEVRVPEQRDALHLPLSWRVKRPRTRIWGGLPDPISRSQLVKSELEEKKSELRHKLKYVPHEYIELIEIARNSTQDRILEMKVMEFFMKVYGYRGKHLGGSRKPDGAIYTVGSPIDYGVIVDTKAYSGGYNLPIGQADEMQRYVEENQTRNKHINPNEWWKVYPSSVTEFKFLFVSGHFKGNYKAQLTRLNHITNCNGAVLSVEELLIGGEMIKAGTLTLEEVRRKFNNGEINF

SEQ ID NO: 73 - protein, 1409 aa, Artificial Sequence
  synthetic
MASSPPKKKRKVSWKDASGWSRMHADPIRPRRPSPARELLPGPQPDRVQPTADRGVSAPAGSPLDGLPARRTVSRTRLPSPPAPSPAFSAGSFSDLLRPFDPSLLDTSLLDSMPAVGTPHTAAAPAEWDEAQSALRAADDPPPTVRVAVTAARPPRAKPAPRRRAAQPSDASPAAQVDLRTLGYSQQQQEKIKPKVRSTVAQHHEALVGHGFTHAHIVALSQHPAALGTVAVTYQHIITALPEATHEDIVGVGKQWSGARALEALLTDAGELRGPPLQLDTGQLVKIAKRGGVTAMEAVHASRNALTGAPLNLTPAQVVAIASHDGGKQALETVQRLLPVLCQDHGLTPDQVVAIASHDGGKQALETVQRLLPVLCQDHGLTPDQVVAIASNIGGKQALETVQRLLPVLCQDHGLTPDQVVAIASNGGGKQALETVQRLLPVLCQDHGLTPDQVVAIASNNGGKQALETVQRLLPVLCQDHGLTPDQVVAIASNIGGKQALETVQRLLPVLCQDHGLTPDQVVAIASNNGGKQALETVQRLLPVLCQDHGLTPDQVVAIASNNGGKQALETVQRLLPVLCQDHGLTPDQVVAIASNIGGKQALETVQRLLPVLCQDHGLTPDQVVAIASNIGGKQALETVQRLLPVLCQDHGLTPDQVVAIASNGGGKQALETVQRLLPVLCQDHGLTPDQVVAIASNIGGKQALETVQRLLPVLCQDHGLTPDQVVAIASNIGGKQALETVQRLLPVLCQDHGLTPDQVVAIASNIGGKQALETVQRLLPVLCQDHGLTPDQVVAIASHDGGKQALETVQRLLPVLCQDHGLTPDQVVAIASNIGGKQALETVQRLLPVLCQDHGLTPDQVVAIASHDGGKQALETVQRLLPVLCQDHGLTPDQVVAIASHDGGKQALETVQRLLPVLCQDHGLTPDQVVAIASHDGGKQALETVQRLLPVLCQDHGLTPDQVVAIASNGGGKQALESIVAQLSRPDPALAALTNDHLVALACLGGRPAMDAVKKGLPHAPELIRRVNRRIGERTSHRVADYAQVVRVLEFFQCHSHPAYAFDEAMTQFGMSRNGLVQLFRRVGVTELEARGGTLPPASQRWDRILQASGMKRAKPSPTSAQTPDQASLHAFADSLERDLDAPSPMHEGDQTRASSRKRSRSDRAVTGPSAQQAVEVRVPEQRDALHLPLSWRVKRPRTRIWGGLPDPISRSQLVKSELEEKKSELRHKLKYVPHEYIELIEIARNSTQDRILEMKVMEFFMKVYGYRGKHLGGSRKPDGAIYTVGSPIDYGVIVDTKAYSGGYNLPIGQADEMQRYVEENQTRNKHINPNEWWKVYPSSVTEFKFLFVSGHFKGNYKAQLTRLNHITNCNGAVLSVEELLIGGEMIKAGTLTLEEVRRKFNNGEINF

SEQ ID NO: 74 - protein, 8 aa, Artificial Sequence
  synthetic
KIAKRGGV

SEQ ID NO: 75 - protein, 8 aa, Artificial Sequence
  synthetic
KIANGGGV

SEQ ID NO: 76 - protein, 8 aa, Artificial Sequence
  synthetic
KIANIGGV

SEQ ID NO: 77 - protein, 8 aa, Artificial Sequence
  synthetic
KIAHDGGV

SEQ ID NO: 78 - protein, 8 aa, Artificial Sequence
  synthetic
KIANNGGV

SEQ ID NO: 79 - protein, 8 aa, Artificial Sequence
  synthetic
KIAKRGGV

SEQ ID NO: 80 - protein, 9 aa, Artificial Sequence
  synthetic
KIASNGGGV

SEQ ID NO: 81 - protein, 9 aa, Artificial Sequence
  synthetic
KIASNIGGV

SEQ ID NO: 82 - protein, 9 aa, Artificial Sequence
  synthetic
KIASHDGGV

SEQ ID NO: 83 - protein, 9 aa, Artificial Sequence
  synthetic
KIASNNGGV

SEQ ID NO: 84 - protein, 8 aa, Artificial Sequence
  synthetic
KIAKRGGV

SEQ ID NO: 85 - protein, 9 aa, Artificial Sequence
  synthetic
KIAKNGGGV

SEQ ID NO: 86 - protein, 9 aa, Artificial Sequence
  synthetic
KIAKNIGGV

SEQ ID NO: 87 - protein, 9 aa, Artificial Sequence
  synthetic
KIAKHDGGV

SEQ ID NO: 88 - protein, 9 aa, Artificial Sequence
  synthetic
KIAKNNGGV

SEQ ID NO: 89 - protein, 8 aa, Artificial Sequence
  synthetic
KIAKRGGV

SEQ ID NO: 90 - protein, 9 aa, Artificial Sequence
  synthetic
KIASNGGGK

SEQ ID NO: 91 - protein, 9 aa, Artificial Sequence
  synthetic
KIASNIGGK

SEQ ID NO: 92 - protein, 9 aa, Artificial Sequence
  synthetic
KIASHDGGK

SEQ ID NO: 93 - protein, 9 aa, Artificial Sequence
  synthetic
KIASNNGGK